European Patent Specification EP 3 315 606 B1, published November 26, 2025. Title: ANTI-HUMAN TRANSFERRIN RECEPTOR ANTIBODY THAT PASSES THROUGH BLOOD-BRAIN BARRIER. Applicant: JCR PHARMACEUTICALS CO., LTD. The sequence listing filed with the application follows.

SEQUENCE LISTING (279 sequences)

SEQ ID NO: 1 - protein, 760 aa, Homo sapiens
MMDQARSAFSNLFGGEPLSYTRFSLARQVDGDNSHVEMKLAVDEEENADNNTKANVTKPKRCSGSICYGTIAVIVFFLIGFMIGYLGYCKGVEPKTECERLAGTESPVREEPGEDFPAARRLYWDDLKRKLSEKLDSTDFTGTIKLLNENSYVPREAGSQKDENLALYVENQFREFKLSKVWRDQHFVKIQVKDSAQNSVIIVDKNGRLVYLVENPGGYVAYSKAATVTGKLVHANFGTKKDFEDLYTPVNGSIVIVRAGKITFAEKVANAESLNAIGVLIYMDQTKFPIVNAELSFFGHAHLGTGDPYTPGFPSFNHTQFPPSRSSGLPNIPVQTISRAAAEKLFGNMEGDCPSDWKTDSTCRMVTSESKNVKLTVSNVLKEIKILNIFGVIKGFVEPDHYVVVGAQRDAWGPGAAKSGVGTALLLKLAQMFSDMVLKDGFQPSRSIIFASWSAGDFGSVGATEWLEGYLSSLHLKAFTYINLDKAVLGTSNFKVSASPLLYTLIEKTMQNVKHPVTGQFLYQDSNWASKVEKLTLDNAAFPFLAYSGIPAVSFCFCEDTDYPYLGTTMDTYKELIERIPELNKVARAAAEVAGQFVIKLTHDVELNLDYERYNSQLLSFVRDLNQYRADIKEMGLSLQWLYSARGDFFRATSRLTTDFGNAEKTDRFVMKKLNDRVMRVEYHFLSPYVSPKESPFRHVFWGSGSHTLPALLENLKLRKQNNGAFNETLFRNQLALATWTIQGAANALSGDVWDIDNEF

SEQ ID NO: 2 - protein, 760 aa, Macaca fascicularis
MMDQARSAFSNLFGGEPLSYTRFSLARQVDGDNSHVEMKLAVDDEENADNNTKANGTKPKRCGGNICYGTIAVIIFFLIGFMIGYLGYCKGVEPKTECERLAGTESPAREEPEEDFPAAPRLYWDDLKRKLSEKLDTTDFTSTIKLLNENLYVPREAGSQKDENLALYIENQFREFKLSKVWRDQHFVKIQVKDSAQNSVIIVDKNGGLVYLVENPGGYVAYSKAATVTGKLVHANFGTKKDFEDLDSPVNGSIVIVRAGKITFAEKVANAESLNAIGVLIYMDQTKFPIVKADLSFFGHAHLGTGDPYTPGFPSFNHTQFPPSQSSGLPNIPVQTISRAAAEKLFGNMEGDCPSDWKTDSTCKMVTSENKSVKLTVSNVLKETKILNIFGVIKGFVEPDHYVVVGAQRDAWGPGAAKSSVGTALLLKLAQMFSDMVLKDGFQPSRSIIFASWSAGDFGSVGATEWLEGYLSSLHLKAFTYINLDKAVLGTSNFKVSASPLLYTLIEKTMQDVKHPVTGRSLYQDSNWASKVEKLTLDNAAFPFLAYSGIPAVSFCFCEDTDYPYLGTTMDTYKELVERIPELNKVARAAAEVAGQFVIKLTHDTELNLDYERYNSQLLLFLRDLNQYRADVKEMGLSLQWLYSARGDFFRATSRLTTDFRNAEKRDKFVMKKLNDRVMRVEYYFLSPYVSPKESPFRHVFWGSGSHTLSALLESLKLRRQNNSAFNETLFRNQLALATWTIQGAANALSGDVWDIDNEF

SEQ ID NO: 3 - protein, 5 aa, Artificial Sequence
  Amino acid sequence of exemplified linker 1
GGGGS

SEQ ID NO: 4 - protein, 6 aa, Artificial Sequence
  Amino acid sequence of exemplified linker 2
GGGGGS

SEQ ID NO: 5 - protein, 5 aa, Artificial Sequence
  Amino acid sequence of exemplified linker 3
SGGGG

SEQ ID NO: 6 - protein, 6 aa, Artificial Sequence
  Amino acid sequence 1 of CDR 1 in the light chain of mouse anti-hTfR antibody No.1
QDVNSA

SEQ ID NO: 7 - protein, 11 aa, Artificial Sequence
  Amino acid sequence 2 of CDR 1 in the light chain of mouse anti-hTfR antibody No.1
KASQDVNSAVA

SEQ ID NO: 8 - protein, 6 aa, Artificial Sequence
  Amino acid sequence 1 of CDR 2 in the light chain of mouse anti-hTfR antibody No.1
WTSTRH

SEQ ID NO: 9 - protein, 7 aa, Artificial Sequence
  Amino acid sequence 2 of CDR 2 in the light chain of mouse anti-hTfR antibody No.1
WTSTRHT

SEQ ID NO: 10 - protein, 9 aa, Artificial Sequence
  Amino acid sequence of CDR 3 in the light chain of mouse anti-hTfR antibody No.1
QQHYSTPRT

SEQ ID NO: 11 - protein, 6 aa, Artificial Sequence
  Amino acid sequence 1 of CDR 1 in the light chain of mouse anti-hTfR antibody No.2
QSISNN

SEQ ID NO: 12 - protein, 11 aa, Artificial Sequence
  Amino acid sequence 2 of CDR 1 in the light chain of mouse anti-hTfR antibody No.2
RASQSISNNLQ

SEQ ID NO: 13 - protein, 6 aa, Artificial Sequence
  Amino acid sequence 1 of CDR 2 in the light chain of mouse anti-hTfR antibody No.2
YASQSI

SEQ ID NO: 14 - protein, 7 aa, Artificial Sequence
  Amino acid sequence 2 of CDR 2 in the light chain of mouse anti-hTfR antibody No.2
YASQSIS

SEQ ID NO: 15 - protein, 9 aa, Artificial Sequence
  Amino acid sequence of CDR 3 in the light chain of mouse anti-hTfR antibody No.2
QQSNSWPRT

SEQ ID NO: 16 - protein, 11 aa, Artificial Sequence
  Amino acid sequence 1 of CDR 1 in the light chain of mouse anti-hTfR antibody No.3
QSLVHSNGNTY

SEQ ID NO: 17 - protein, 16 aa, Artificial Sequence
  Amino acid sequence 2 of CDR 1 in the light chain of mouse anti-hTfR antibody No.3
RSSQSLVHSNGNTYLH

SEQ ID NO: 18 - protein, 6 aa, Artificial Sequence
  Amino acid sequence 1 of CDR 2 in the light chain of mouse anti-hTfR antibody No.3
KVSNRF

SEQ ID NO: 19 - protein, 7 aa, Artificial Sequence
  Amino acid sequence 2 of CDR 2 in the light chain of mouse anti-hTfR antibody No.3
KVSNRFS

SEQ ID NO: 20 - protein, 9 aa, Artificial Sequence
  Amino acid sequence of CDR 3 in the light chain of mouse anti-hTfR antibody No.3
SQSTHVPWT

SEQ ID NO: 21 - protein, 5 aa, Artificial Sequence
  Amino acid sequence 1 of CDR 1 in the light chain of mouse anti-hTfR antibody No.4
SNVNY

SEQ ID NO: 22 - protein, 10 aa, Artificial Sequence
  Amino acid sequence 2 of CDR 1 in the light chain of mouse anti-hTfR antibody No.4
SASSNVNYMH

SEQ ID NO: 23 - protein, 6 aa, Artificial Sequence
  Amino acid sequence 1 of CDR 2 in the light chain of mouse anti-hTfR antibody No.4
DTSKLA

SEQ ID NO: 24 - protein, 7 aa, Artificial Sequence
  Amino acid sequence 2 of CDR 2 in the light chain of mouse anti-hTfR antibody No.4
DTSKLAS

SEQ ID NO: 25 - protein, 9 aa, Artificial Sequence
  Amino acid sequence of CDR 3 in the light chain of mouse anti-hTfR antibody No.4
FQGNGNPYT

SEQ ID NO: 26 - protein, 5 aa, Artificial Sequence
  Amino acid sequence 1 of CDR 1 in the light chain of mouse anti-hTfR antibody No.5
SSISS

SEQ ID NO: 27 - protein, 10 aa, Artificial Sequence
  Amino acid sequence 2 of CDR 1 in the light chain of mouse anti-hTfR antibody No.5
SASSSISSIH

SEQ ID NO: 28 - protein, 6 aa, Artificial Sequence
  Amino acid sequence 1 of CDR 2 in the light chain of mouse anti-hTfR antibody No.5
DTSTLA

SEQ ID NO: 29 - protein, 7 aa, Artificial Sequence
  Amino acid sequence 2 of CDR 2 in the light chain of mouse anti-hTfR antibody No.5
DTSTLAS

SEQ ID NO: 30 - protein, 8 aa, Artificial Sequence
  Amino acid sequence of CDR 3 in the light chain of mouse anti-hTfR antibody No.5
HQRSSYPT

SEQ ID NO: 31 - protein, 6 aa, Artificial Sequence
  Amino acid sequence 1 of CDR 1 in the light chain of mouse anti-hTfR antibody No.6
QEISGY

SEQ ID NO: 32 - protein, 11 aa, Artificial Sequence
  Amino acid sequence 2 of CDR 1 in the light chain of mouse anti-hTfR antibody No.6
RASQEISGYLS

SEQ ID NO: 33 - protein, 6 aa, Artificial Sequence
  Amino acid sequence 1 of CDR 2 in the light chain of mouse anti-hTfR antibody No.6
AASTLD

SEQ ID NO: 34 - protein, 7 aa, Artificial Sequence
  Amino acid sequence 2 of CDR 2 in the light chain of mouse anti-hTfR antibody No.6
AASTLDS

SEQ ID NO: 35 - protein, 9 aa, Artificial Sequence
  Amino acid sequence of CDR 3 in the light chain of mouse anti-hTfR antibody No.6
LQYSSYPRT

SEQ ID NO: 36 - protein, 5 aa, Artificial Sequence
  Amino acid sequence 1 of CDR 1 in the light chain of mouse anti-hTfR antibody No.7
SSVNY

SEQ ID NO: 37 - protein, 10 aa, Artificial Sequence
  Amino acid sequence 2 of CDR 1 in the light chain of mouse anti-hTfR antibody No.7
SASSSVNYIH

SEQ ID NO: 38 - protein, 6 aa, Artificial Sequence
  Amino acid sequence 1 of CDR 2 in the light chain of mouse anti-hTfR antibody No.7
QTSNLA

SEQ ID NO: 39 - protein, 7 aa, Artificial Sequence
  Amino acid sequence 2 of CDR 2 in the light chain of mouse anti-hTfR antibody No.7
QTSNLAS

SEQ ID NO: 40 - protein, 9 aa, Artificial Sequence
  Amino acid sequence of CDR 3 in the light chain of mouse anti-hTfR antibody No.7
HQWSSYPWT

SEQ ID NO: 41 - protein, 5 aa, Artificial Sequence
  Amino acid sequence 1 of CDR 1 in the light chain of mouse anti-hTfR antibody No.8
SSVSY

SEQ ID NO: 42 - protein, 10 aa, Artificial Sequence
  Amino acid sequence 2 of CDR 1 in the light chain of mouse anti-hTfR antibody No.8
SASSSVSYMH

SEQ ID NO: 43 - protein, 6 aa, Artificial Sequence
  Amino acid sequence 1 of CDR 2 in the light chain of mouse anti-hTfR antibody No.8
GTSNLA

SEQ ID NO: 44 - protein, 7 aa, Artificial Sequence
  Amino acid sequence 2 of CDR 2 in the light chain of mouse anti-hTfR antibody No.8
GTSNLAS

SEQ ID NO: 45 - protein, 9 aa, Artificial Sequence
  Amino acid sequence of CDR 3 in the light chain of mouse anti-hTfR antibody No.8
HQWSSYPWT

SEQ ID NO: 46 - protein, 5 aa, Artificial Sequence
  Amino acid sequence 1 of CDR 1 in the light chain of mouse anti-hTfR antibody No.9
SSVSL

SEQ ID NO: 47 - protein, 10 aa, Artificial Sequence
  Amino acid sequence 2 of CDR 1 in the light chain of mouse anti-hTfR antibody No.9
SASSSVSLMF

SEQ ID NO: 48 - protein, 6 aa, Artificial Sequence
  Amino acid sequence 1 of CDR 2 in the light chain of mouse anti-hTfR antibody No.9
FTSYRA

SEQ ID NO: 49 - protein, 7 aa, Artificial Sequence
  Amino acid sequence 2 of CDR 2 in the light chain of mouse anti-hTfR antibody No.9
FTSYRAS

SEQ ID NO: 50 - protein, 9 aa, Artificial Sequence
  Amino acid sequence of CDR 3 in the light chain of mouse anti-hTfR antibody No.9
QQWTSDPPT

SEQ ID NO: 51 - protein, 6 aa, Artificial Sequence
  Amino acid sequence 1 of CDR 1 in the light chain of mouse anti-hTfR antibody No.10
QEISGY

SEQ ID NO: 52 - protein, 11 aa, Artificial Sequence
  Amino acid sequence 2 of CDR 1 in the light chain of mouse anti-hTfR antibody No.10
RPSQEISGYLS

SEQ ID NO: 53 - protein, 6 aa, Artificial Sequence
  Amino acid sequence 1 of CDR 2 in the light chain of mouse anti-hTfR antibody No.10
AASTLD

SEQ ID NO: 54 - protein, 7 aa, Artificial Sequence
  Amino acid sequence 2 of CDR 2 in the light chain of mouse anti-hTfR antibody No.10
AASTLDS

SEQ ID NO: 55 - protein, 9 aa, Artificial Sequence
  Amino acid sequence of CDR 3 in the light chain of mouse anti-hTfR antibody No.10
LQYASYPRT

SEQ ID NO: 56 - protein, 6 aa, Artificial Sequence
  Amino acid sequence 1 of CDR 1 in the light chain of mouse anti-hTfR antibody No.11
QSIRNY

SEQ ID NO: 57 - protein, 11 aa, Artificial Sequence
  Amino acid sequence 2 of CDR 1 in the light chain of mouse anti-hTfR antibody No.11
RASQSIRNYLH

SEQ ID NO: 58 - protein, 6 aa, Artificial Sequence
  Amino acid sequence 1 of CDR 2 in the light chain of mouse anti-hTfR antibody No.11
YASQSI

SEQ ID NO: 59 - protein, 7 aa, Artificial Sequence
  Amino acid sequence 2 of CDR 2 in the light chain of mouse anti-hTfR antibody No.11
YASQSIS

SEQ ID NO: 60 - protein, 9 aa, Artificial Sequence
  Amino acid sequence of CDR 3 in the light chain of mouse anti-hTfR antibody No.11
QQTNSWPYT

SEQ ID NO: 61 - protein, 6 aa, Artificial Sequence
  Amino acid sequence 1 of CDR 1 in the light chain of mouse anti-hTfR antibody No.12
HDVKTA

SEQ ID NO: 62 - protein, 11 aa, Artificial Sequence
  Amino acid sequence 2 of CDR 1 in the light chain of mouse anti-hTfR antibody No.12
KASHDVKTAVA

SEQ ID NO: 63 - protein, 6 aa, Artificial Sequence
  Amino acid sequence 1 of CDR 2 in the light chain of mouse anti-hTfR antibody No.12
WSSTRH

SEQ ID NO: 64 - protein, 7 aa, Artificial Sequence
  Amino acid sequence 2 of CDR 2 in the light chain of mouse anti-hTfR antibody No.12
WSSTRHT

SEQ ID NO: 65 - protein, 9 aa, Artificial Sequence
  Amino acid sequence of CDR 3 in the light chain of mouse anti-hTfR antibody No.12
QQHFSTPLT

SEQ ID NO: 66 - protein, 6 aa, Artificial Sequence
  Amino acid sequence 1 of CDR 1 in the light chain of mouse anti-hTfR antibody No.13
QSIRNY

SEQ ID NO: 67 - protein, 11 aa, Artificial Sequence
  Amino acid sequence 2 of CDR 1 in the light chain of mouse anti-hTfR antibody No.13
RASQSIRNYLH

SEQ ID NO: 68 - protein, 6 aa, Artificial Sequence
  Amino acid sequence 1 of CDR 2 in the light chain of mouse anti-hTfR antibody No.13
YASQSI

SEQ ID NO: 69 - protein, 7 aa, Artificial Sequence
  Amino acid sequence 2 of CDR 2 in the light chain of mouse anti-hTfR antibody No.13
YASQSIS

SEQ ID NO: 70 - protein, 9 aa, Artificial Sequence
  Amino acid sequence of CDR 3 in the light chain of mouse anti-hTfR antibody No.13
QQTNSWPYT

SEQ ID NO: 71 - protein, 5 aa, Artificial Sequence
  Amino acid sequence 1 of CDR 1 in the light chain of mouse anti-hTfR antibody No.14
SNINS

SEQ ID NO: 72 - protein, 10 aa, Artificial Sequence
  Amino acid sequence 2 of CDR 1 in the light chain of mouse anti-hTfR antibody No.14
SASSNINSIH

SEQ ID NO: 73 - protein, 6 aa, Artificial Sequence
  Amino acid sequence 1 of CDR 2 in the light chain of mouse anti-hTfR antibody No.14
DTSNLA

SEQ ID NO: 74 - protein, 7 aa, Artificial Sequence
  Amino acid sequence 2 of CDR 2 in the light chain of mouse anti-hTfR antibody No.14
DTSNLAS

SEQ ID NO: 75 - protein, 9 aa, Artificial Sequence
  Amino acid sequence of CDR 3 in the light chain of mouse anti-hTfR antibody No.14
HQRSGYPFT

SEQ ID NO: 76 - protein, 5 aa, Artificial Sequence
  Amino acid sequence 1 of CDR 1 in the heavy chain of mouse anti-hTfR antibody No.1
NYGMS

SEQ ID NO: 77 - protein, 8 aa, Artificial Sequence
  Amino acid sequence 2 of CDR 1 in the heavy chain of mouse anti-hTfR antibody No.1
GLTFSNYG

SEQ ID NO: 78 - protein, 8 aa, Artificial Sequence
  Amino acid sequence 1 of CDR 2 in the heavy chain of mouse anti-hTfR antibody No.1
INTNGGST

SEQ ID NO: 79 - protein, 17 aa, Artificial Sequence
  Amino acid sequence 2 of CDR 2 in the heavy chain of mouse anti-hTfR antibody No.1
NINTNGGSTYYPDSVKG

SEQ ID NO: 80 - protein, 7 aa, Artificial Sequence
  Amino acid sequence 1 of CDR 3 in the heavy chain of mouse anti-hTfR antibody No.1
NRYDEDY

SEQ ID NO: 81 - protein, 9 aa, Artificial Sequence
  Amino acid sequence 2 of CDR 3 in the heavy chain of mouse anti-hTfR antibody No.1
TNNRYDEDY

SEQ ID NO: 82 - protein, 5 aa, Artificial Sequence
  Amino acid sequence 1 of CDR 1in the heavy chain of mouse anti-hTfR antibody No.2
DYVMH

SEQ ID NO: 83 - protein, 8 aa, Artificial Sequence
  Amino acid sequence 2 of CDR 1 in the heavy chain of mouse anti-hTfR antibody No.2
GYTFTDYV

SEQ ID NO: 84 - protein, 8 aa, Artificial Sequence
  Amino acid sequence 1 of CDR 2 in the heavy chain of mouse anti-hTfR antibody No.2
ISTYYGHG

SEQ ID NO: 85 - protein, 17 aa, Artificial Sequence
  Amino acid sequence 2 of CDR 2 in the heavy chain of mouse anti-hTfR antibody No.2
VISTYYGHGSYNQRFKG

SEQ ID NO: 86 - protein, 14 aa, Artificial Sequence
  Amino acid sequence 1 of CDR 3 in the heavy chain of mouse anti-hTfR antibody No.2
GGYGSSSLAGNFDV

SEQ ID NO: 87 - protein, 16 aa, Artificial Sequence
  Amino acid sequence 2 of CDR 3 in the heavy chain of mouse anti-hTfR antibody No.2
VRGGYGSSSLAGNFDV

SEQ ID NO: 88 - protein, 5 aa, Artificial Sequence
  Amino acid sequence 1 of CDR 1 in the heavy chain of mouse anti-hTfR antibody No.3
NYWLG

SEQ ID NO: 89 - protein, 8 aa, Artificial Sequence
  Amino acid sequence 2 of CDR 1 in the heavy chain of mouse anti-hTfR antibody No.3
GYSFTNYW

SEQ ID NO: 90 - protein, 8 aa, Artificial Sequence
  Amino acid sequence 1 of CDR 2 in the heavy chain of mouse anti-hTfR antibody No.3
IYPGGDYP

SEQ ID NO: 91 - protein, 17 aa, Artificial Sequence
  Amino acid sequence 2 of CDR 2 in the heavy chain of mouse anti-hTfR antibody No.3
DIYPGGDYPTYSEKFKV

SEQ ID NO: 92 - protein, 9 aa, Artificial Sequence
  Amino acid sequence 1 of CDR 3 in the heavy chain of mouse anti-hTfR antibody No.3
SGNYDEVAY

SEQ ID NO: 93 - protein, 11 aa, Artificial Sequence
  Amino acid sequence 2 of CDR 3 in the heavy chain of mouse anti-hTfR antibody No.3
ARSGNYDEVAY

SEQ ID NO: 94 - protein, 5 aa, Artificial Sequence
  Amino acid sequence 1 of CDR 1 in the heavy chain of mouse anti-hTfR antibody No.4
NYLIE

SEQ ID NO: 95 - protein, 8 aa, Artificial Sequence
  Amino acid sequence 2 of CDR 1 in the heavy chain of mouse anti-hTfR antibody No.4
GYAFTNYL

SEQ ID NO: 96 - protein, 8 aa, Artificial Sequence
  Amino acid sequence 1 of CDR 2 in the heavy chain of mouse anti-hTfR antibody No.4
INPGSGGI

SEQ ID NO: 97 - protein, 16 aa, Artificial Sequence
  Amino acid sequence 2 of CDR 2 in the heavy chain of mouse anti-hTfR antibody No.4
INPGSGGIIYNEKFTD

SEQ ID NO: 98 - protein, 13 aa, Artificial Sequence
  Amino acid sequence 1 of CDR 3 in the heavy chain of mouse anti-hTfR antibody No.4
SNYYGTTYWHFDV

SEQ ID NO: 99 - protein, 15 aa, Artificial Sequence
  Amino acid sequence 2 of CDR 3 in the heavy chain of mouse anti-hTfR antibody No.4
ARSNYYGTTYWHFDV

SEQ ID NO: 100 - protein, 5 aa, Artificial Sequence
  Amino acid sequence 1 of CDR 1 in the heavy chain of mouse anti-hTfR antibody No.5
NFVIH

SEQ ID NO: 101 - protein, 8 aa, Artificial Sequence
  Amino acid sequence 2 of CDR 1 in the heavy chain of mouse anti-hTfR antibody No.5
GYTFTNFV

SEQ ID NO: 102 - protein, 8 aa, Artificial Sequence
  Amino acid sequence 1 of CDR 2 in the heavy chain of mouse anti-hTfR antibody No.5
FNPHKNGA

SEQ ID NO: 103 - protein, 16 aa, Artificial Sequence
  Amino acid sequence 2 of CDR 2 in the heavy chain of mouse anti-hTfR antibody No.5
FNPHKNGAEYNEKFQV

SEQ ID NO: 104 - protein, 9 aa, Artificial Sequence
  Amino acid sequence 1 of CDR 3 in the heavy chain of mouse anti-hTfR antibody No.5
SFYYYSMDY

SEQ ID NO: 105 - protein, 11 aa, Artificial Sequence
  Amino acid sequence 2 of CDR 3 in the heavy chain of mouse anti-hTfR antibody No.5
ARSFYYYSMDY

SEQ ID NO: 106 - protein, 5 aa, Artificial Sequence
  Amino acid sequence 1 of CDR 1 in the heavy chain of mouse anti-hTfR antibody No.6
TYGVY

SEQ ID NO: 107 - protein, 8 aa, Artificial Sequence
  Amino acid sequence 2 of CDR 1 in the heavy chain of mouse anti-hTfR antibody No.6
GFSLSTYG

SEQ ID NO: 108 - protein, 7 aa, Artificial Sequence
  Amino acid sequence of CDR 2 in the heavy chain of mouse anti-hTfR antibody No.6
IWGDGST

SEQ ID NO: 109 - protein, 4 aa, Artificial Sequence
  Amino acid sequence 1 of CDR 3 in the heavy chain of mouse anti-hTfR antibody No.6
PDDV

SEQ ID NO: 110 - protein, 6 aa, Artificial Sequence
  Amino acid sequence 2 of CDR 3 in the heavy chain of mouse anti-hTfR antibody No.6
AKPDDV

SEQ ID NO: 111 - protein, 5 aa, Artificial Sequence
  Amino acid sequence 1 of CDR 1 in the heavy chain of mouse anti-hTfR antibody No.7
NYFMS

SEQ ID NO: 112 - protein, 8 aa, Artificial Sequence
  Amino acid sequence 2 of CDR 1 in the heavy chain of mouse anti-hTfR antibody No.7
GITFRNYF

SEQ ID NO: 113 - protein, 8 aa, Artificial Sequence
  Amino acid sequence 1 of CDR 2 in the heavy chain of mouse anti-hTfR antibody No.7
ISSAGGYT

SEQ ID NO: 114 - protein, 16 aa, Artificial Sequence
  Amino acid sequence 2 of CDR 2 in the heavy chain of mouse anti-hTfR antibody No.7
ISSAGGYTYYADSVKG

SEQ ID NO: 115 - protein, 11 aa, Artificial Sequence
  Amino acid sequence 1 of CDR 3 in the heavy chain of mouse anti-hTfR antibody No.7
QEVPYPYAMDY

SEQ ID NO: 116 - protein, 13 aa, Artificial Sequence
  Amino acid sequence 2 of CDR 3 in the heavy chain of mouse anti-hTfR antibody No.7
ARQEVPYPYAMDY

SEQ ID NO: 117 - protein, 5 aa, Artificial Sequence
  Amino acid sequence 1 of CDR 1 in the heavy chain of mouse anti-hTfR antibody No.8
TYGVS

SEQ ID NO: 118 - protein, 8 aa, Artificial Sequence
  Amino acid sequence 2 of CDR 1 in the heavy chain of mouse anti-hTfR antibody No.8
GFSLTTYG

SEQ ID NO: 119 - protein, 7 aa, Artificial Sequence
  Amino acid sequence of CDR 2 in the heavy chain of mouse anti-hTfR antibody No.8
IWGDGST

SEQ ID NO: 120 - protein, 4 aa, Artificial Sequence
  Amino acid sequence 1 of CDR 3 in the heavy chain of mouse anti-hTfR antibody No.8
PDDY

SEQ ID NO: 121 - protein, 6 aa, Artificial Sequence
  Amino acid sequence 2 of CDR 3 in the heavy chain of mouse anti-hTfR antibody No.8
AKPDDY

SEQ ID NO: 122 - protein, 5 aa, Artificial Sequence
  Amino acid sequence 1 of CDR 1 in the heavy chain of mouse anti-hTfR antibody No.9
NYGVS

SEQ ID NO: 123 - protein, 8 aa, Artificial Sequence
  Amino acid sequence 2 of CDR 1 in the heavy chain of mouse anti-hTfR antibody No.9
GYTFTNYG

SEQ ID NO: 124 - protein, 8 aa, Artificial Sequence
  Amino acid sequence 1 of CDR 2 in the heavy chain of mouse anti-hTfR antibody No.9
IYTFTGEA

SEQ ID NO: 125 - protein, 16 aa, Artificial Sequence
  Amino acid sequence 2 of CDR 2 in the heavy chain of mouse anti-hTfR antibody No.9
IYTFTGEATYIDDFRG

SEQ ID NO: 126 - protein, 8 aa, Artificial Sequence
  Amino acid sequence 1 of CDR 3 in the heavy chain of mouse anti-hTfR antibody No.9
RNGAWFED

SEQ ID NO: 127 - protein, 10 aa, Artificial Sequence
  Amino acid sequence 2 of CDR 3 in the heavy chain of mouse anti-hTfR antibody No.9
SRRNGAWFED

SEQ ID NO: 128 - protein, 5 aa, Artificial Sequence
  Amino acid sequence 1 of CDR 1 in the heavy chain of mouse anti-hTfR antibody No.10
NYAMS

SEQ ID NO: 129 - protein, 8 aa, Artificial Sequence
  Amino acid sequence 2 of CDR 1 in the heavy chain of mouse anti-hTfR antibody No.10
GITFRNYA

SEQ ID NO: 130 - protein, 8 aa, Artificial Sequence
  Amino acid sequence 1 of CDR 2 in the heavy chain of mouse anti-hTfR antibody No.10
ISSYGGYT

SEQ ID NO: 131 - protein, 16 aa, Artificial Sequence
  Amino acid sequence 2 of CDR 2 in the heavy chain of mouse anti-hTfR antibody No.10
ISSYGGYTYYADSVKG

SEQ ID NO: 132 - protein, 11 aa, Artificial Sequence
  Amino acid sequence 1 of CDR 3 in the heavy chain of mouse anti-hTfR antibody No.10
QEVPYPYPMDN

SEQ ID NO: 133 - protein, 13 aa, Artificial Sequence
  Amino acid sequence 2 of CDR 3 in the heavy chain of mouse anti-hTfR antibody No.10
ARQEVPYPYPMDN

SEQ ID NO: 134 - protein, 5 aa, Artificial Sequence
  Amino acid sequence 1 of CDR 1 in the heavy chain of mouse anti-hTfR antibody No.11
IYWIN

SEQ ID NO: 135 - protein, 8 aa, Artificial Sequence
  Amino acid sequence 2 of CDR 1 in the heavy chain of mouse anti-hTfR antibody No.11
GYAFSIYW

SEQ ID NO: 136 - protein, 8 aa, Artificial Sequence
  Amino acid sequence 1 of CDR 2 in the heavy chain of mouse anti-hTfR antibody No.11
IYPGNGDT

SEQ ID NO: 137 - protein, 16 aa, Artificial Sequence
  Amino acid sequence 2 of CDR 2 in the heavy chain of mouse anti-hTfR antibody No.11
IYPGNGDTNYNGKFKG

SEQ ID NO: 138 - protein, 9 aa, Artificial Sequence
  Amino acid sequence 1 of CDR 3 in the heavy chain of mouse anti-hTfR antibody No.11
WGDDYAMDF

SEQ ID NO: 139 - protein, 11 aa, Artificial Sequence
  Amino acid sequence 2 of CDR 3 in the heavy chain of mouse anti-hTfR antibody No.11
GRWGDDYAMDF

SEQ ID NO: 140 - protein, 5 aa, Artificial Sequence
  Amino acid sequence 1 of CDR 1 in the heavy chain of mouse anti-hTfR antibody No.12
NYLIE

SEQ ID NO: 141 - protein, 8 aa, Artificial Sequence
  Amino acid sequence 2 of CDR 1 in the heavy chain of mouse anti-hTfR antibody No.12
GYVFINYL

SEQ ID NO: 142 - protein, 8 aa, Artificial Sequence
  Amino acid sequence 1 of CDR 2 in the heavy chain of mouse anti-hTfR antibody No.12
IHSGSGGT

SEQ ID NO: 143 - protein, 16 aa, Artificial Sequence
  Amino acid sequence 2 of CDR 2 in the heavy chain of mouse anti-hTfR antibody No.12
IHSGSGGTNYNDNFKD

SEQ ID NO: 144 - protein, 10 aa, Artificial Sequence
  Amino acid sequence 1 of CDR 3 in the heavy chain of mouse anti-hTfR antibody No.12
RNFGNYYFDY

SEQ ID NO: 145 - protein, 12 aa, Artificial Sequence
  Amino acid sequence 2 of CDR 3 in the heavy chain of mouse anti-hTfR antibody No.12
ARRNFGNYYFDY

SEQ ID NO: 146 - protein, 5 aa, Artificial Sequence
  Amino acid sequence 1 of CDR 1 in the heavy chain of mouse anti-hTfR antibody No.13
IYWIN

SEQ ID NO: 147 - protein, 8 aa, Artificial Sequence
  Amino acid sequence 2 of CDR 1 in the heavy chain of mouse anti-hTfR antibody No.13
GYAFSIYW

SEQ ID NO: 148 - protein, 8 aa, Artificial Sequence
  Amino acid sequence 1 of CDR 2 in the heavy chain of mouse anti-hTfR antibody No.13
IYPGNGDT

SEQ ID NO: 149 - protein, 16 aa, Artificial Sequence
  Amino acid sequence 2 of CDR 2 in the heavy chain of mouse anti-hTfR antibody No.13
IYPGNGDTNYNGKFKG

SEQ ID NO: 150 - protein, 9 aa, Artificial Sequence
  Amino acid sequence 1 of CDR 3 in the heavy chain of mouse anti-hTfR antibody No.13
WGDDYAMDF

SEQ ID NO: 151 - protein, 11 aa, Artificial Sequence
  Amino acid sequence 2 of CDR 3 in the heavy chain of mouse anti-hTfR antibody No.13
GRWGDDYAMDF

SEQ ID NO: 152 - protein, 5 aa, Artificial Sequence
  Amino acid sequence 1 of CDR 1 in the heavy chain of mouse anti-hTfR antibody No.14
GYVIH

SEQ ID NO: 153 - protein, 8 aa, Artificial Sequence
  Amino acid sequence 2 of CDR 1 in the heavy chain of mouse anti-hTfR antibody No.14
GYAFTGYV

SEQ ID NO: 154 - protein, 8 aa, Artificial Sequence
  Amino acid sequence 1 of CDR 2 in the heavy chain of mouse anti-hTfR antibody No.14
LNPHKDDS

SEQ ID NO: 155 - protein, 16 aa, Artificial Sequence
  Amino acid sequence 2 of CDR 2 in the heavy chain of mouse anti-hTfR antibody No.14
LNPHKDDSEYNEKFRG

SEQ ID NO: 156 - protein, 9 aa, Artificial Sequence
  Amino acid sequence 1 of CDR 3 in the heavy chain of mouse anti-hTfR antibody No.14
GYYYYSMDY

SEQ ID NO: 157 - protein, 11 aa, Artificial Sequence
  Amino acid sequence 2 of CDR 3 in the heavy chain of mouse anti-hTfR antibody No.14
ARGYYYYSMDY

SEQ ID NO: 158 - protein, 107 aa, Artificial Sequence
  Amino acid sequence 1 of the variable region of light chain of humanized anti-hTfR antibody No.1
DIVMTQSPDSLAVSLGERATINCKASQDVNSAVAWYQQKPGQPPKLLIYWTSTRHTGVPDRFSGSGSGTDFTLTISSLQAEDVAVYYCQQHYSTPRTFGGGTKLEIK

SEQ ID NO: 159 - protein, 107 aa, Artificial Sequence
  Amino acid sequence 2 of the variable region of light chain of humanized anti-hTfR antibody No.1
DIQMTQSPSSLSASVGDRVTITCKASQDVNSAVAWYQQKPGKAPKLLLYWTSTRHTGVPSRFSGSGSGTDYTLTISSLQPEDFATYYCQQHYSTPRTFGGGTKVEIK

SEQ ID NO: 160 - protein, 107 aa, Artificial Sequence
  Amino acid sequence 3 of the variable region of light chain of humanized anti-hTfR antibody No.1
DIQVTQSPSFLSASVGDRVTITCKASQDVNSAVAWYQQKPGKAPKLLIYWTSTRHTGVPSRFSGSGSGTEFTLTISSLQPEDFATYYCQQHYSTPRTFGGGTKVEIK

SEQ ID NO: 161 - protein, 107 aa, Artificial Sequence
  Amino acid sequence 4 of the variable region of light chain of humanized anti-hTfR antibody No.1
DIQMTQSPSSLSASVGDRVTITCKASQDVNSAVAWYQQKPGKAPKLLIYWTSTRHTGVPSRFSGSGSGTDFTLTISSLQPEDFATYYCQQHYSTPRTFGGGTKVEIK

SEQ ID NO: 162 - protein, 107 aa, Artificial Sequence
  Amino acid sequence 5 of the variable region of light chain of humanized anti-hTfR antibody No.1
DIQMTQSPSSVSASVGDRVTITCKASQDVNSAVAWYQQKPGKAPKLLIYWTSTRHTGVPSRFSGSGSGTDFTLTISSLQPEDFATYYCQQHYSTPRTFGQGTKVEIK

SEQ ID NO: 163 - protein, 107 aa, Artificial Sequence; identical to SEQ ID NO: 162
  Amino acid sequence 6 of the variable region of light chain of humanized anti-hTfR antibody No.1

SEQ ID NO: 164 - protein, 214 aa, Artificial Sequence
  Amino acid sequence of the light chain of humanized anti-hTfR antibody No.1 containing amino acid sequence 6 as the variable region
DIQVTQSPSFLSASVGDRVTITCKASQDVNSAVAWFQQKPGKAPKLLIYWTSTRHTGVPDRFSGSGSGTVYTLTISSLQPEDFATYYCQQHYSTPRTFGGGTKVEIKRTVAAPSVFIFPPSDEQLKSGTASVVCLLNNFYPREAKVQWKVDNALQSGNSQESVTEQDSKDSTYSLSSTLTLSKADYEKHKVYACEVTHQGLSSPVTKSFNRGEC

SEQ ID NO: 165 - DNA, 725 bp, Artificial Sequence
  Nucleotide sequence encoding the amino acid sequence of the light chain of humanized anti-hTfR antibody No.1 containing amino acid sequence 6 as the variable region, synthetic sequence
acgcgtgccgccaccatgggctggagctggattctgctgttcctcctgagcgtgacagcaggagtgcacagcgacatccaggtcacacagtcaccaagttttctgagcgcaagcgtgggcgacagggtcactatcacatgcaaggcaagccaggacgtgaactccgcagtggcctggttccagcagaagccagggaaagcacccaagctgctgatctattggacctctacaaggcacaccggtgtcccagatcggttctcaggttccggcagcggaacagtgtatactctgaccatttccagcctgcagcctgaagacttcgctacttactattgccagcagcattactccaccccaagaacatttggcggagggactaaagtggagatcaagaggaccgtggccgctccctccgtcttcatttttccccctagcgacgaacagctgaagagtggcacagcctcagtggtctgtctgctgaacaatttctaccctagggaggctaaagtgcagtggaaggtcgataacgcactgcagtctggaaatagtcaggagtcagtgacagaacaggactccaaagatagcacttattctctgtctagtacactgactctgagcaaggccgattacgaaaagcacaaagtgtatgcttgcgaagtcacccatcaggggctgtcatcaccagtcaccaagtcattcaatagaggcgagtgctaagcggccgc

SEQ ID NO: 166 - protein, 116 aa, Artificial Sequence
  Amino acid sequence 1 of the variable region of the heavy chain of humanized anti-hTfR antibody No.1
EVQLLESGGGLVQPGGSLRLSCAASGFTFSNYGMSWVRQAPGKGLEWVSNINTNGGSTYYPDSVKGRFTISRDNSKNTLYLQMNSLRAEDTAVYYCAKNRYDEDYWGQGTLVTVSS

SEQ ID NO: 167 - protein, 116 aa, Artificial Sequence
  Amino acid sequence 2 of the variable region of the heavy chain of humanized anti-hTfR antibody No.1
EVQLVESGGGLVQPGGSLRLSCAASGFTFSNYGMSWVRQAPGKGLEWVSNINTNGGSTYYPDSVKGRFTISRDNSKNTLYLQMNSLRAEDTAVYYCAKNRYDEDYWGQGTLVTVSS

SEQ ID NO: 168 - protein, 116 aa, Artificial Sequence
  Amino acid sequence 3 of the variable region of the heavy chain of humanized anti-hTfR antibody No.1
EVQLVESGGGLVQPGGSLRLSCSASGFTFSNYGMSWVRQAPGKGLEYVSNINTNGGSTYYPDSVKGRFTISRDNSKNTLYLQMSSLRAEDTAVYYCVKNRYDEDYWGQGTLVTVSS

SEQ ID NO: 169 - protein, 116 aa, Artificial Sequence
  Amino acid sequence 4 of the variable region of the heavy chain of humanized anti-hTfR antibody No.1
EVQLVESGGGLVQPGGSLRLSCAASGFTFSNYGMSWVRQAPGKGLEWVANINTNGGSTYYPDSVKGRFTISRDNAKNSLYLQMNSLRAEDTAVYYCARNRYDEDYWGQGTLVTVSS

SEQ ID NO: 170 - protein, 116 aa, Artificial Sequence
  Amino acid sequence 5 of the variable region of the heavy chain of humanized anti-hTfR antibody No.1
EVQLVESGGGLVQPGGSLRLSCAASGFTFSNYGMSWVRQAPGKGLVWVSNINTNGGSTYYPDSVKGRFTISRDNAKNTLYLQMNSLRAEDTAVYYCARNRYDEDYWGQGTLVTVSS

SEQ ID NO: 171 - protein, 116 aa, Artificial Sequence
  Amino acid sequence 6 of the variable region of the heavy chain of humanized anti-hTfR antibody No.1
EVQLVESGGGLVQPGGSLRLSCAASGLTFSNYGMSWVRQAPGKGLELVANINTNGGSTYYPDSVKGRFTISRDNAKNSLYLQMNSLRAEDTAVYYCTNNRYDEDYWGQGTLVTVSS

SEQ ID NO: 172 - protein, 446 aa, Artificial Sequence
  Amino acid sequence of the heavy chain of humanized anti-hTfR antibody No.1 containing amino acid sequence 6 as the variable region
EVQLVESGGGLVQPGGSLRLSCAASGLTFSNYGMSWVRQAPGKGLELVANINTNGGSTYYPDSVKGRFTISRDNAKNSLYLQMNSLRAEDTAVYYCTNNRYDEDYWGQGTLVTVSSASTKGPSVFPLAPSSKSTSGGTAALGCLVKDYFPEPVTVSWNSGALTSGVHTFPAVLQSSGLYSLSSVVTVPSSSLGTQTYICNVNHKPSNTKVDKKVEPKSCDKTHTCPPCPAPELLGGPSVFLFPPKPKDTLMISRTPEVTCVVVDVSHEDPEVKFNWYVDGVEVHNAKTKPREEQYNSTYRVVSVLTVLHQDWLNGKEYKCKVSNKALPAPIEKTISKAKGQPREPQVYTLPPSRDELTKNQVSLTCLVKGFYPSDIAVEWESNGQPENNYKTTPPVLDSDGSFFLYSKLTVDKSRWQQGNVFSCSVMHEALHNHYTQKSLSLSPGK

SEQ ID NO: 173 - DNA, 1421 bp, Artificial Sequence
  Nucleotide sequence encoding the amino acid sequence of the heavy chain of humanized anti-hTfR antibody No.1 containing amino acid sequence 6 as the variable region, synthetic sequence
acgcgtgccgccaccatgggctggagctggattctgctgttcctcctgagcgtgacagcaggagtgcacagcgaagtgcagctggtcgaatcagggggggggctggtgcagcctggaggcagcctgagactgtcctgcgccgcttctggcttgacctttagcaactacgggatgtcctgggtgcggcaggctcctggcaagggactggagttggtggccaacatcaataccaacggcggaagtacatactatcccgattcagtgaagggccggttcaccatcagcagggacaacgccaagaacagcctgtatctgcagatgaactctctgagggccgaggatacagccgtgtactattgcactaacaaccggtacgacgaggactattggggccagggcaccctggtgacagtgtctagcgcctctaccaagggcccaagcgtgtttcctctggctccatcctctaaatccacctctggcggcacagccgctctgggctgtctggtgaaggattacttcccagagcccgtgacagtgtcttggaacagcggcgccctgacctccggcgtgcacacatttcctgctgtgctgcagagctccggcctgtacagcctgtctagcgtggtgaccgtgccatcctctagcctgggcacccagacatatatctgcaacgtgaatcacaagcccagcaatacaaaggtggataagaaggtggagccaaagtcctgtgacaagacccacacatgccccccttgtcctgctccagagctgctgggaggaccaagcgtgttcctgtttccacccaagcccaaggataccctgatgatctctcggaccccagaggtgacatgcgtggtggtggatgtgagccacgaggaccccgaggtgaagttcaactggtatgtggacggcgtggaggtgcacaatgctaagaccaagcccagggaggagcagtacaactccacctatagagtggtgtctgtgctgacagtgctgcaccaggattggctgaacggcaaggagtataagtgcaaggtgtccaataaggccctgcccgctcctatcgagaagaccatctctaaggccaagggccagcccagagagcctcaggtgtacacactgcctccatcccgggatgagctgaccaagaaccaggtgtctctgacatgtctggtcaagggcttctatccctctgacatcgccgtggagtgggagagcaatggccagcctgagaacaattacaagaccacaccccctgtgctggattccgacggctctttctttctgtatagcaagctgaccgtggacaagtcccggtggcagcagggcaacgtgttcagctgttccgtgatgcacgaagctctgcataatcactatactcagaaatccctgtcactgtcacctggtaaataagcggccgc

SEQ ID NO: 174 - protein, 107 aa, Artificial Sequence
  Amino acid sequence 1 of the variable region of the light chain of humanized anti-hTfR antibody No.2
EIVMTQSPATLSVSPGERATLSCRASQSISNNLQWYQQKPGQAPRLLIYYASQSISGIPARFSGSGSGTEFTLTISSLQSEDFAVYYCQQSNSWPRTFGQGTKVDIK

SEQ ID NO: 175 - protein, 107 aa, Artificial Sequence
  Amino acid sequence 2 of the variable region of the light chain of humanized anti-hTfR antibody No.2
EIVMTQSPATLSLSPGERATLSCRASQSISNNLQWYQQKPGQAPRLLIYYASQSISGIPARFSGSGSGTDFTLTISSLEPEDFAVYYCQQSNSWPRTFGGGTKVEIK

SEQ ID NO: 176 - protein, 107 aa, Artificial Sequence
  Amino acid sequence 3 of the variable region of the light chain of humanized anti-hTfR antibody No.2
EIVLTQSPDFQSVTPKEKVTITCRASQSISNNLQWYQQKPDQSPKLLIKYASQSISGVPSRFSGSGSGTDFTLTINSLEAEDAATYYCQQSNSWPRTFGQGTKVEIK

SEQ ID NO: 177 - protein, 107 aa, Artificial Sequence
  Amino acid sequence 4 of the variable region of the light chain of humanized anti-hTfR antibody No.2
EIVLTQSPATLSLSPGERATLSCRASQSISNNLQWYQQKPGQAPRLLIYYASQSISGIPARFSGSGSGTDFTLTISSLEPEDFAVYYCQQSNSWPRTFGQGTKVEIK

SEQ ID NO: 178 - protein, 107 aa, Artificial Sequence
  Amino acid sequence 5 of the variable region of the light chain of humanized anti-hTfR antibody No.2
DIQMTQSPSSLSASVGDRVTITCRASQSISNNLQWYQQKPGKAPKLLIYYASQSISGVPSRFSGSGSGTDFTLTISSLQPEDFATYYCQQSNSWPRTFGGGTKVEIK

SEQ ID NO: 179 - protein, 107 aa, Artificial Sequence
  Amino acid sequence 6 of the variable region of the light chain of humanized anti-hTfR antibody No.2
EIVLTQSPDFQSVTPKEKVTITCRASQSISNNLQWYQQKPDQSPKLLIKYASQSISGIPSRFSGSGSGTDFTLTINSLEAEDAATYLCQQSNSWPRTFGQGTKVEIK

SEQ ID NO: 180 - protein, 214 aa, Artificial Sequence
  Amino acid sequence of the light chain of humanized anti-hTfR antibody No.2 containing amino acid sequence 6 as the variable region
EIVLTQSPDFQSVTPKEKVTITCRASQSISNNLQWYQQKPDQSPKLLIKYASQSISGIPSRFSGSGSGTDFTLTINSLEAEDAATYLCQQSNSWPRTFGQGTKVEIKRTVAAPSVFIFPPSDEQLKSGTASVVCLLNNFYPREAKVQWKVDNALQSGNSQESVTEQDSKDSTYSLSSTLTLSKADYEKHKVYACEVTHQGLSSPVTKSFNRGEC

SEQ ID NO: 181 - DNA, 725 bp, Artificial Sequence
  Nucleotide sequence encoding the amino acid sequence of the light chain of humanized anti-hTfR antibody No.2 containing amino acid sequence 6 as the variable region, synthetic sequence
acgcgtgccgccaccatgggctggagctggattctgctgttcctcctgagcgtgacagcaggagtgcacagcgaaattgtgctgacccagtctcccgatttccagtccgtgacccccaaggagaaagtcaccatcacatgcagagcatcacagtccattagcaacaatctgcagtggtaccagcagaagccagaccagagccccaagctgctgatcaaatatgcctctcagagtatttcaggcataccttctaggttctccggtagcggctctggaaccgactttactctgaccatcaacagtctggaggctgaagatgccgctacatacttgtgccagcagagtaattcatggcctaggacctttggccaggggacaaaggtggagatcaaaaggactgtggcagccccaagtgtcttcatttttcccccttcagacgaacagctgaagagcggcacagcatctgtggtctgtctgctgaacaatttctacccacgggaggctaaggtgcagtggaaagtcgataacgcactgcagtccggaaatagccaggagtctgtgactgaacaggacagtaaggattcaacctattccctgtccagcacactgactctgagcaaagccgattacgagaagcacaaagtgtatgcttgcgaagtcacacatcaggggctgtctagtcccgtgactaagtcttttaataggggtgaatgttaagcggccgc

SEQ ID NO: 182 - protein, 120 aa, Artificial Sequence
  Amino acid sequence 1 of the variable region of the heavy chain of humanized anti-hTfR antibody No.2
QVQLVQSGAEVKKPGASVKVSCKASGYTFTDYVMHWVRQAPGQGLEWMGVISTYYGHGSYNQRFKGRVTMTRDTSTSTVYMELSSLRSEDTAVYYCARGGYGSSSLAGNFDVWGQGTLVT

SEQ ID NO: 183 - protein, 120 aa, Artificial Sequence
  Amino acid sequence 2 of the variable region of the heavy chain of humanized anti-hTfR antibody No.2
QVQLVQSGAEVKKPGASVKVSCKASGYTFTDYVMHWVRQAPGQRLEWMGVISTYYGHGSYNQRFKGRVTITRDTSASTAYMELSSLRSEDTAVYYCARGGYGSSSLAGNFDVWGQGTLVT

SEQ ID NO: 184 - protein, 120 aa, Artificial Sequence
  Amino acid sequence 3 of the variable region of the heavy chain of humanized anti-hTfR antibody No.2
QVQLVQSGAEVKKPGASVKVSCKASGYTFTDYVMHWVRQAPGQGLEWMGVISTYYGHGSYNQRFKGRVTMTTDTSTSAAYMELRSLRSDDTAVYYCASGGYGSSSLAGNFDVWGQGTLVT

SEQ ID NO: 185 - protein, 120 aa, Artificial Sequence
  Amino acid sequence 4 of the variable region of the heavy chain of humanized anti-hTfR antibody No.2
QVQLVQSGAEVKKPGASVKVSCKASGYTFTDYVMHWVRQAPGQGLEWMGVISTYYGHGSYNQRFKGRVTMTRDTSISTAYMELSRLRSDDTAVYYCARGGYGSSSLAGNFDVWGQGTTVT

SEQ ID NO: 186 - protein, 120 aa, Artificial Sequence
  Amino acid sequence 5 of the variable region of the heavy chain of humanized anti-hTfR antibody No.2
QVQLVQSGAEVKKPGSSVKVSCKASGGTFSDYVMHWVRQAPGQGLEWMGVISTYYGHGSYNQRFKGRVTITADKSTSTAYMELSSLRSEDTAVYYCARGGYGSSSLAGNFDVWGQGTVVT

SEQ ID NO: 187 - protein, 120 aa, Artificial Sequence
  Amino acid sequence 6 of the variable region of the heavy chain of humanized anti-hTfR antibody No.2
QVQLVQSGAEVKKPGASVKVSCKASGYTFTDYVMHWVRQAPGQGLEWIGVISTYYGHGSYNQRFKGRATMTVDKSISTAYMELVRLRSDDTAVYYCVRGGYGSSSLAGNFDVWGQGTTVT

SEQ ID NO: 188 - protein, 453 aa, Artificial Sequence
  Amino acid sequence of the heavy chain of humanized anti-hTfR antibody No.2 containing amino acid sequence 6 as the variable region
QVQLVQSGAEVKKPGASVKVSCKASGYTFTDYVMHWVRQAPGQGLEWIGVISTYYGHGSYNQRFKGRATMTVDKSISTAYMELVRLRSDDTAVYYCVRGGYGSSSLAGNFDVWGQGTTVTVSSASTKGPSVFPLAPSSKSTSGGTAALGCLVKDYFPEPVTVSWNSGALTSGVHTFPAVLQSSGLYSLSSVVTVPSSSLGTQTYICNVNHKPSNTKVDKKVEPKSCDKTHTCPPCPAPELLGGPSVFLFPPKPKDTLMISRTPEVTCVVVDVSHEDPEVKFNWYVDGVEVHNAKTKPREEQYNSTYRVVSVLTVLHQDWLNGKEYKCKVSNKALPAPIEKTISKAKGQPREPQVYTLPPSRDELTKNQVSLTCLVKGFYPSDIAVEWESNGQPENNYKTTPPVLDSDGSFFLYSKLTVDKSRWQQGNVFSCSVMHEALHNHYTQKSLSLSPGK

SEQ ID NO: 189 - DNA, 1442 bp, Artificial Sequence
  Nucleotide sequence encoding the amino acid sequence of the heavy chain of humanized anti-hTfR antibody No.2 containing amino acid sequence 6 as the variable region, synthetic sequence
acgcgtgccgccaccatgggctggagctggattctgctgttcctcctgagcgtgacagcaggagtgcacagccaggtgcagctggtccagtcaggagccgaagtgaaaaagcccggagcctcagtcaaagtgtcttgtaaagcatcaggttatacatttacagactacgtcatgcactgggtgaggcaggcacctggacagggtctggaatggatcggcgtgatctccacttactatggccatggaagctacaaccagagattcaagggcagggcgacaatgactgtagacaaatcaatttccactgcttatatggagctggtaaggctgcggtccgacgataccgctgtgtactattgcgtacgaggaggatacggctccagctctctggctggtaatttcgatgtgtgggggcagggtaccacagtcaccgtgagttcagcaagcacaaagggcccatctgtgtttccactggccccctccagcaaaagcacctctgggggtacagccgctctgggatgtctggtgaaggattatttcccagagccagtcaccgtgtcctggaacagcggagccctgacatctggagtccacacttttccagctgtgctgcagtctagtgggctgtactccctgtcatccgtggtcactgtccccagctctagtctgggtacccagacatatatctgcaacgtgaatcacaagccatctaataccaaagtcgacaagaaagtggaacccaagtcctgtgataaaactcatacctgccccccttgtcctgcaccagagctgctgggaggaccatccgtgttcctgtttccacccaagcctaaagacaccctgatgattagccgaactcccgaagtcacctgcgtggtcgtggacgtgtctcacgaggaccctgaagtcaagtttaactggtacgtggatggcgtcgaggtgcataatgctaagacaaaaccccgagaggaacagtacaacagtacatatcgtgtcgtgtcagtgctgaccgtcctgcatcaggactggctgaacgggaaggaatataagtgcaaagtgtccaataaggcactgcccgcccctatcgagaaaaccattagcaaggccaaaggacagcctagggaaccacaggtgtacacactgcctccatcccgggacgagctgactaagaaccaggtcagcctgacctgtctggtgaaaggcttctatccttcagatatcgctgtggagtgggaaagtaatggacagccagagaacaattacaagactaccccccctgtgctggactctgatgggagtttctttctgtattctaagctgaccgtggataaaagtcggtggcagcagggtaatgtctttagttgttcagtgatgcacgaagcactgcacaaccactacacccagaaatcactgtcactgtcaccagggaaataagcggccgc

SEQ ID NO: 190 - protein, 112 aa, Artificial Sequence
  Amino acid sequence 1 of the variable region of the light chain of humanized anti-hTfR antibody No.3
DVVMTQSPLSLPVTLGQPASISCRSSQSLVHSNGNTYLHWFQQRPGQSPRRLIYKVSNRFSGVPDRFSGSGSGTDFTLKISRVEAEDVGVYYCSQSTHVPWTFGGGTKVEIK

SEQ ID NO: 191 - protein, 112 aa, Artificial Sequence
  Amino acid sequence 2 of the variable region of the light chain of humanized anti-hTfR antibody No.3
DIVMTQTPLSLSVTPGQPASISCRSSQSLVHSNGNTYLHWYLQKPGQSPQLLIYKVSNRFSGVPDRFSGSGSGTDFTLKISRVEAEDVGVYYCSQSTHVPWTFGQGTKVEIK

SEQ ID NO: 192 - protein, 112 aa, Artificial Sequence
  Amino acid sequence 3 of the variable region of the light chain of humanized anti-hTfR antibody No.3
DIVMTQTPLSSPVTLGQPASISCRSSQSLVHSNGNTYLHWLQQRPGQPPRLLIYKVSNRFSGVPDRFSGSGAGTDFTLKISRVEAEDVGVYYCSQSTHVPWTFGQGTKLEIK

SEQ ID NO: 193 - protein, 112 aa, Artificial Sequence
  Amino acid sequence 4 of the variable region of the light chain of humanized anti-hTfR antibody No.3
DIVMTQSPLSLPVTPGEPASISCRSSQSLVHSNGNTYLHWYLQKPGQSPQLLIYKVSNRFSGVPDRFSGSGSGTDFTLKISRVEAEDVGVYYCSQSTHVPWTFGQGTKVEIK

SEQ ID NO: 194 - protein, 112 aa, Artificial Sequence
  Amino acid sequence 5 of the variable region of the light chain of humanized anti-hTfR antibody No.3
DIVMTQTPLSLPVTPGEPASISCRSSQSLVHSNGNTYLHWYLQKPGQSPQLLIYKVSNRFSGVPDRFSGSGSGTDFTLKISRVEAEDVGVYYCSQSTHVPWTFGQGTRLEIK

SEQ ID NO: 195 - protein, 112 aa, Artificial Sequence
  Amino acid sequence 6 of the variable region of the light chain of humanized anti-hTfR antibody No.3
DIVMTQTPLSLSVTPGQPASISCRSSQSLVHSNGNTYLHWYLQKPGQSPQLLIYKVSNRFSGVPDRFSGSGSGTDFTLKISRVEAEDVGVFFCSQSTHVPWTFGQGTKVEIK

SEQ ID NO: 196 - protein, 219 aa, Artificial Sequence
  Amino acid sequence of the light chain of humanized anti-hTfR antibody No.3 containing amino acid sequence 2 as the variable region
DIVMTQTPLSLSVTPGQPASISCRSSQSLVHSNGNTYLHWYLQKPGQSPQLLIYKVSNRFSGVPDRFSGSGSGTDFTLKISRVEAEDVGVYYCSQSTHVPWTFGQGTKVEIKRTVAAPSVFIFPPSDEQLKSGTASVVCLLNNFYPREAKVQWKVDNALQSGNSQESVTEQDSKDSTYSLSSTLTLSKADYEKHKVYACEVTHQGLSSPVTKSFNRGEC

SEQ ID NO: 197 - DNA, 740 bp, Artificial Sequence
  Nucleotide sequence encoding the amino acid sequence of the light chain of humanized anti-hTfR antibody No.3 containing amino acid sequence 2 as the variable region, synthetic sequence
acgcgtgccgccaccatgggctggagctggattctgctgttcctcctgagcgtgacagcaggagtgcacagcgacatcgtgatgacccagactcccctgagcctgagcgtgacacctggccagcctgccagcatcagctgcagaagctctcagagcctggtgcacagcaacggcaacacctacctgcactggtatctgcagaagcccggccagagccctcagctgctgatctacaaggtgtccaacagattcagcggcgtgcccgacagattctccggcagcggctctggcaccgacttcaccctgaagatttccagagtggaagccgaggacgtgggcgtgtactactgcagccagagcacccacgtgccctggacattcggccagggcaccaaggtggaaatcaagagaaccgtggccgctcccagcgtgttcatcttcccacctagcgacgagcagctgaagtccggcacagcctctgtcgtgtgcctgctgaacaacttctacccccgcgaggccaaggtgcagtggaaggtggacaacgccctgcagagcggcaacagccaggaaagcgtgaccgagcaggactccaaggacagcacctacagcctgagcagcaccctgaccctgagcaaggccgactacgagaagcacaaggtgtacgcctgcgaagtgacccaccagggcctgtctagccccgtgaccaagagcttcaacagaggcgagtgctaagcggccgc

SEQ ID NO: 198 - protein, 219 aa, Artificial Sequence
  Amino acid sequence of the light chain of humanized anti-hTfR antibody No.3 containing amino acid sequence 4 as the variable region
DIVMTQSPLSLPVTPGEPASISCRSSQSLVHSNGNTYLHWYLQKPGQSPQLLIYKVSNRFSGVPDRFSGSGSGTDFTLKISRVEAEDVGVYYCSQSTHVPWTFGQGTKVEIKRTVAAPSVFIFPPSDEQLKSGTASVVCLLNNFYPREAKVQWKVDNALQSGNSQESVTEQDSKDSTYSLSSTLTLSKADYEKHKVYACEVTHQGLSSPVTKSFNRGEC

SEQ ID NO: 199 - DNA, 740 bp, Artificial Sequence
  Nucleotide sequence encoding the amino acid sequence of the light chain of humanized anti-hTfR antibody No.3 containing amino acid sequence 4 as the variable region, synthetic sequence
acgcgtgccgccaccatgggctggagctggattctgctgttcctcctgagcgtgacagcaggagtgcacagcgacatcgtgatgacccagagccccctgagcctgcctgtgacacctggcgagcctgccagcatcagctgcagatctagccagagcctggtgcacagcaacggcaacacctacctgcactggtatctgcagaagcccggccagagccctcagctgctgatctacaaggtgtccaacagattcagcggcgtgcccgacagattctccggcagcggctctggcaccgacttcaccctgaagatctccagagtggaagccgaggacgtgggcgtgtactactgcagccagagcacccacgtgccctggacattcggccagggcaccaaggtggaaatcaagagaaccgtggccgctcccagcgtgttcatcttcccacctagcgacgagcagctgaagtccggcacagcctctgtcgtgtgcctgctgaacaacttctacccccgcgaggccaaggtgcagtggaaggtggacaacgccctgcagagcggcaacagccaggaaagcgtgaccgagcaggactccaaggacagcacctacagcctgagcagcaccctgaccctgagcaaggccgactacgagaagcacaaggtgtacgcctgcgaagtgacccaccagggcctgtctagccccgtgaccaagagcttcaacagaggcgagtgctaagcggccgc

SEQ ID NO: 200 - protein, 219 aa, Artificial Sequence
  Amino acid sequence of the light chain of humanized anti-hTfR antibody No.3 containing amino acid sequence 5 as the variable region
DIVMTQTPLSLPVTPGEPASISCRSSQSLVHSNGNTYLHWYLQKPGQSPQLLIYKVSNRFSGVPDRFSGSGSGTDFTLKISRVEAEDVGVYYCSQSTHVPWTFGQGTRLEIKRTVAAPSVFIFPPSDEQLKSGTASVVCLLNNFYPREAKVQWKVDNALQSGNSQESVTEQDSKDSTYSLSSTLTLSKADYEKHKVYACEVTHQGLSSPVTKSFNRGEC

SEQ ID NO: 201 - DNA, 740 bp, Artificial Sequence
  Nucleotide sequence encoding the amino acid sequence of the light chain of humanized anti-hTfR antibody No.3 containing amino acid sequence 5 as the variable region, synthetic sequence
acgcgtgccgccaccatgggctggagctggattctgctgttcctcctgagcgtgacagcaggagtgcacagcgacatcgtgatgacccagacacccctgagcctgcctgtgacacctggcgagcctgccagcatcagctgcagatctagccagagcctggtgcacagcaacggcaacacctacctgcactggtatctgcagaagcccggccagagccctcagctgctgatctacaaggtgtccaacagattcagcggcgtgcccgacagattctccggcagcggctctggcaccgacttcaccctgaagatctccagagtggaagccgaggacgtgggcgtgtactactgcagccagagcacccacgtgccctggacattcggccagggcaccaggctggaaatcaagagaaccgtggccgctcccagcgtgttcatcttcccacctagcgacgagcagctgaagtccggcacagcctctgtcgtgtgcctgctgaacaacttctacccccgcgaggccaaggtgcagtggaaggtggacaacgccctgcagagcggcaacagccaggaaagcgtgaccgagcaggactccaaggacagcacctacagcctgagcagcaccctgaccctgagcaaggccgactacgagaagcacaaggtgtacgcctgcgaagtgacccaccagggcctgtctagccccgtgaccaagagcttcaacagaggcgagtgctaagcggccgc

SEQ ID NO: 202 - protein, 219 aa, Artificial Sequence
  Amino acid sequence of the light chain of humanized anti-hTfR antibody No.3 containing amino acid sequence 6 as the variable region
DIVMTQTPLSLSVTPGQPASISCRSSQSLVHSNGNTYLHWYLQKPGQSPQLLIYKVSNRFSGVPDRFSGSGSGTDFTLKISRVEAEDVGVFFCSQSTHVPWTFGQGTKVEIKRTVAAPSVFIFPPSDEQLKSGTASVVCLLNNFYPREAKVQWKVDNALQSGNSQESVTEQDSKDSTYSLSSTLTLSKADYEKHKVYACEVTHQGLSSPVTKSFNRGEC

SEQ ID NO: 203 - DNA, 740 bp, Artificial Sequence
  Nucleotide sequence encoding the amino acid sequence of the light chain of humanized anti-hTfR antibody No.3 containing amino acid sequence 6 as the variable region, synthetic sequence
acgcgtgccgccaccatgggctggagctggattctgctgttcctcctgagcgtgacagcaggagtgcacagcgacatcgtgatgacccagactcccctgagcctgagcgtgacacctggccagcctgccagcatcagctgcagatccagccagagcctggtgcacagcaacggcaacacctacctgcactggtatctgcagaagcccggccagagccctcagctgctgatctacaaggtgtccaacagattcagcggcgtgcccgacagattctccggcagcggctctggcaccgacttcaccctgaagatttccagagtggaagccgaggacgtgggcgtgttcttctgcagccagagcacccacgtgccctggacattcggccagggcaccaaggtggaaatcaagagaaccgtggccgctcccagcgtgttcatcttcccacctagcgacgagcagctgaagtccggcacagcctctgtcgtgtgcctgctgaacaacttctacccccgcgaggccaaggtgcagtggaaggtggacaacgccctgcagagcggcaacagccaggaaagcgtgaccgagcaggactccaaggacagcacctacagcctgagcagcaccctgaccctgagcaaggccgactacgagaagcacaaggtgtacgcctgcgaagtgacccaccagggcctgtctagccccgtgaccaagagcttcaacagaggcgagtgctaagcggccgc

SEQ ID NO: 204 - protein, 118 aa, Artificial Sequence
  Amino acid sequence 1 of the variable region of the heavy chain of humanized anti-hTfR antibody No.3
QVQLVQSGAEVKKPGASVKVSCKASGYTFTNYWLGWVRQAPGQGLEWMGDIYPGGDYPTYSEKFKVRVTMTRDTSTSTVYMELSSLRSEDTAVYYCARSGNYDEVAYWGQGTLVTVSS

SEQ ID NO: 205 - protein, 118 aa, Artificial Sequence
  Amino acid sequence 2 of the variable region of the heavy chain of humanized anti-hTfR antibody No.3
EVQLVQSGAEVKKPGESLKISCKGSGYSFTNYWLGWVRQMPGKGLEWMGDIYPGGDYPTYSEKFKVQVTISADKSISTAYLQWSSLKASDTAMYYCARSGNYDEVAYWGQGTLVTVSS

SEQ ID NO: 206 - protein, 118 aa, Artificial Sequence
  Amino acid sequence 3 of the variable region of the heavy chain of humanized anti-hTfR antibody No.3
QVQLVQSGAEVKKPGASVKVSCKASGYTFTNYWLGWVRQAPGQGLEWMGDIYPGGDYPTYSEKFKVRVTMTRDTSISTAYMELSRLRSDDTAVYYCARSGNYDEVAYWGQGTTVTVSS

SEQ ID NO: 207 - protein, 118 aa, Artificial Sequence
  Amino acid sequence 4 of the variable region of the heavy chain of humanized anti-hTfR antibody No.3
QVQLVQSGAEVKKPGASVKVSCKASGYTFTNYWLGWVRQAPGQRLEWMGDIYPGGDYPTYSEKFKVRVTITRDTSASTAYMELSSLRSEDTAVYYCARSGNYDEVAYWGQGTLVTVSS

SEQ ID NO: 208 - protein, 118 aa, Artificial Sequence
  Amino acid sequence 5 of the variable region of the heavy chain of humanized anti-hTfR antibody No.3
QVQLVQSGAEVKKPGSSVKVSCKASGGTFSNYWLGWVRQAPGQGLEWMGDIYPGGDYPTYSEKFKVRVTITADKSTSTAYMELSSLRSEDTAVYYCARSGNYDEVAYWGQGTVVTVSS

SEQ ID NO: 209 - protein, 118 aa, Artificial Sequence
  Amino acid sequence 6 of the variable region of the heavy chain of humanized anti-hTfR antibody No.3
EVQLVQSGAEVKKPGESLKISCKGSGYSFMNYWLGWVRQMPGKGLEWIGDIYPGGDYPTYSEKFKVKAIISADTSISTVYLQLSSLKASDTAMYFCARSGNYDEVAYWGQGTLVTVSS

SEQ ID NO: 210 - protein, 448 aa, Artificial Sequence
  Amino acid sequence of the heavy chain of humanized anti-hTfR antibody No.3 containing amino acid sequence 2 as the variable region
EVQLVQSGAEVKKPGESLKISCKGSGYSFTNYWLGWVRQMPGKGLEWMGDIYPGGDYPTYSEKFKVQVTISADKSISTAYLQWSSLKASDTAMYYCARSGNYDEVAYWGQGTLVTVSSASTKGPSVFPLAPSSKSTSGGTAALGCLVKDYFPEPVTVSWNSGALTSGVHTFPAVLQSSGLYSLSSVVTVPSSSLGTQTYICNVNHKPSNTKVDKKVEPKSCDKTHTCPPCPAPELLGGPSVFLFPPKPKDTLMISRTPEVTCVVVDVSHEDPEVKFNWYVDGVEVHNAKTKPREEQYNSTYRVVSVLTVLHQDWLNGKEYKCKVSNKALPAPIEKTISKAKGQPREPQVYTLPPSRDELTKNQVSLTCLVKGFYPSDIAVEWESNGQPENNYKTTPPVLDSDGSFFLYSKLTVDKSRWQQGNVFSCSVMHEALHNHYTQKSLSLSPGK

SEQ ID NO: 211 - DNA, 1427 bp, Artificial Sequence
  Nucleotide sequence encoding the amino acid sequence of the heavy chain of humanized anti-hTfR antibody No.3 containing amino acid sequence 2 as the variable region, synthetic sequence
acgcgtgccgccaccatgggctggagctggattctgctgttcctcctgagcgtgacagcaggagtgcacagcgaggtgcaactagtgcagtctggagcagaggtgaaaaagcccggggagtctctgaagatttcctgtaagggttctggatacagctttaccaactactggctgggatgggtgcgccagatgcccgggaaaggcctggagtggatgggggacatctaccccggcggagactaccctacatacagcgagaagttcaaggtccaggtcaccatctcagccgacaagtccatcagcaccgcctacctgcagtggagcagcctgaaggcctcggacaccgccatgtattactgtgcgagatcaggcaattacgacgaagtggcctactggggccaaggaaccctggtcaccgtctcctcagctagcaccaagggcccatcggtcttccccctggcaccctcctccaagagcacctctgggggcacagcggccctgggctgcctggtcaaggactacttccccgaaccggtgacggtgtcgtggaactcaggcgccctgaccagcggcgtgcacaccttcccggctgtcctacagtcctcaggactctactccctcagcagcgtggtgaccgtgccctccagcagcttgggcacccagacctacatctgcaacgtgaatcacaagcccagcaacaccaaggtggacaagaaagttgagcccaaatcttgtgacaaaactcacacgtgcccaccgtgcccagcacctgaactcctgggaggtccgtcagtcttcctcttccccccaaaacccaaggacaccctcatgatctcccggacccctgaggtcacatgcgtggtggtggacgtgagccacgaagaccctgaggtcaagttcaactggtacgtggacggcgtggaggtgcataatgccaagacaaagccgcgggaggagcagtacaacagcacgtaccgggtggtcagcgtcctcaccgtcctgcaccaggactggctgaatggcaaggagtacaagtgcaaggtctccaacaaagccctcccagcccccatcgagaaaaccatctccaaagccaaagggcagccccgagaaccacaggtgtacaccctgcccccatcccgggatgagctgaccaagaaccaggtcagcctgacctgcctggtcaaaggcttctatcccagcgacatcgccgtggagtgggagagcaatgggcagccggagaacaactacaagaccacgcctcccgtgctggactccgacggctccttcttcctctacagcaagctcaccgtggacaagagcaggtggcagcaggggaacgtcttctcatgctccgtgatgcatgaggctctgcacaaccactacacgcagaagagcctctccctgtctccgggtaaataagcggccgc

SEQ ID NO: 212 - protein, 445 aa, Artificial Sequence
  Amino acid sequence of the heavy chain (IgG4) of humanized anti-hTfR antibody No.3 containing amino acid sequence 2 as the variable region
EVQLVQSGAEVKKPGESLKISCKGSGYSFTNYWLGWVRQMPGKGLEWMGDIYPGGDYPTYSEKFKVQVTISADKSISTAYLQWSSLKASDTAMYYCARSGNYDEVAYWGQGTLVTVSSASTKGPSVFPLAPCSRSTSESTAALGCLVKDYFPEPVTVSWNSGALTSGVHTFPAVLQSSGLYSLSSVVTVPSSSLGTKTYTCNVDHKPSNTKVDKRVESKYGPPCPPCPAPEFLGGPSVFLFPPKPKDTLMISRTPEVTCVVVDVSQEDPEVQFNWYVDGVEVHNAKTKPREEQFNSTYRVVSVLTVLHQDWLNGKEYKCKVSNKGLPSSIEKTISKAKGQPREPQVYTLPPSQEEMTKNQVSLTCLVKGFYPSDIAVEWESNGQPENNYKTTPPVLDSDGSFFLYSRLTVDKSRWQEGNVFSCSVMHEALHNHYTQKSLSLSPGK

SEQ ID NO: 213 - DNA, 1418 bp, Artificial Sequence
  Nucleotide sequence encoding the amino acid sequence of the heavy chain (IgG4) of humanized anti-hTfR antibody No.3 containing amino acid sequence 2 as the variable region, synthetic sequence
acgcgtgccgccaccatgggctggagctggattctgctgttcctcctgagcgtgacagcaggagtgcacagcgaggtgcaactagtgcagtctggagcagaggtgaaaaagcccggggagtctctgaagatttcctgtaagggttctggatacagctttaccaactactggctgggatgggtgcgccagatgcccgggaaaggcctggagtggatgggggacatctaccccggcggagactaccctacatacagcgagaagttcaaggtccaggtcaccatctcagccgacaagtccatcagcaccgcctacctgcagtggagcagcctgaaggcctcggacaccgccatgtattactgtgcgagatcaggcaattacgacgaagtggcctactggggccaaggaaccctggtcaccgtctcctcagctagcaccaagggcccatcggtcttccccctggcgccctgctccaggagcacctccgagagcacagccgccctgggctgcctggtcaaggactacttccccgaaccggtgacggtgtcgtggaactcaggcgccctgaccagcggcgtgcacaccttcccggctgtcctacagtcctcaggactctactccctcagcagcgtggtgaccgtgccctccagcagcttgggcacgaagacctacacctgcaacgtagatcacaagcccagcaacaccaaggtggacaagagagttgagtccaaatatggtcccccatgcccaccatgcccagcacctgagttcctggggggtccatcagtcttcctgttccccccaaaacccaaggacactctcatgatctcccggacccctgaggtcacgtgcgtggtggtggacgtgagccaggaagaccccgaggtccagttcaactggtacgtggatggcgtggaggtgcataatgccaagacaaagccgcgggaggagcagttcaacagcacgtaccgtgtggtcagcgtcctcaccgtcctgcaccaggactggctgaacggcaaggagtacaagtgcaaggtctccaacaaaggcctcccgtcctccatcgagaaaaccatctccaaagccaaagggcagccccgagagccacaggtgtacaccctgcccccatcccaggaggagatgaccaagaaccaggtcagcctgacctgcctggtcaaaggcttctaccccagcgacatcgccgtggagtgggagagcaatgggcagccggagaacaactacaagaccacgcctcccgtgctggactccgacggctccttcttcctctacagcaggctcaccgtggacaagagcaggtggcaggaggggaatgtcttctcatgctccgtgatgcatgaggctctgcacaaccactacacacagaagagcctctccctgtctccgggtaaataagcggccgc

SEQ ID NO: 214 - DNA, 43 bp, Artificial Sequence
  Primer hTfR5', synthetic sequence
ccgacgcgtcgccaccatgatggatcaagctagatcagcattc

SEQ ID NO: 215 - DNA, 59 bp, Artificial Sequence
  Primer hTfR3', synthetic sequence
ataatgcggccgcttaatgatgatgatgatgatgaaactcattgtcaatgtcccaaacg

SEQ ID NO: 216 - DNA, 20 bp, Artificial Sequence
  Primer Hyg-Sfi5', synthetic sequence
gaggccgcctcggcctctga

SEQ ID NO: 217 - DNA, 29 bp, Artificial Sequence
  Primer Hyg-BstX3', synthetic sequence
aaccatcgtgatgggtgctattcctttgc

SEQ ID NO: 218 - protein, 108 aa, Artificial Sequence
  Amino acid sequence of the variable region of the light chain of anti-hTfR antibody No.1
DIVLTQSSKFMSTSVGDRVSITCKASQDVNSAVAWFQQKPGQSPKLLIYWTSTRHTGVPDRFTGSGSGTVYTLTISSVQAEDLALYYCQQHYSTPRTFGGGTKLEIKR

SEQ ID NO: 219 - protein, 116 aa, Artificial Sequence
  Amino acid sequence of the variable region of the heavy chain of anti-hTfR antibody No.1
EVQLQESGGGLVQPGGSLKLSCAASGLTFSNYGMSWIRQTPDKRLELVANINTNGGSTYYPDSVKGRFTISRDNAKNTLYLQMNSLKSEDTAIYYCTNNRYDEDYWGQGTSVTVSS

SEQ ID NO: 220 - protein, 108 aa, Artificial Sequence
  Amino acid sequence of the variable region of the light chain of anti-hTfR antibody No.2
DIVLTQSPATLSVTPGDSVSLSCRASQSISNNLQWYQQKSHESPRLLIKYASQSISGIPSRFSGSGSGTDFTLSINSVETEDFGMYFCQQSNSWPRTFGAGTKLELKR

SEQ ID NO: 221 - protein, 123 aa, Artificial Sequence
  Amino acid sequence of the variable region of the heavy chain of anti-hTfR antibody No.2
EVQLQESGAELVRPGVSVKISCKGSGYTFTDYVMHWVRQSHAKSLEWIGVISTYYGHGSYNQRFKGKATMTVDKSSSTAYLELVRLTSEDSAIYYCVRGGYGSSSLAGNFDVWGAGTTVTVSS

SEQ ID NO: 222 - protein, 113 aa, Artificial Sequence
  Amino acid sequence of the variable region of the light chain of anti-hTfR antibody No.3
DIVMTQTTLSLPVSLGDQASISCRSSQSLVHSNGNTYLHWYLQKPGQSPKLLIYKVSNRFSGVPDRFSGSGSGTDFTLKISRVEAEDLGVFFCSQSTHVPWTFGGGTKLEIKR

SEQ ID NO: 223 - protein, 118 aa, Artificial Sequence
  Amino acid sequence of the variable region of the heavy chain of anti-hTfR antibody No.3
EVQLQESGAELVRPGTSVKISCKASGYTFMNYWLGWVKQRPGHGLEWIGDIYPGGDYPTYSEKFKVKAILTADTSSSSVYLHLSSLTSEDSAVYFCARSGNYDEVAYWGQGTLVTVST

SEQ ID NO: 224 - protein, 106 aa, Artificial Sequence
  Amino acid sequence of the variable region of the light chain of anti-hTfR antibody No.4
DIVLTQTPAIMSASPGEKVTMTCSASSNVNYMHWYQQKSSTSPKLWIYDTSKLASGVPGRFSGSGSGNSYSLTISSMEAEDVATYYCFQGNGNPYTFGGGTKLEIK

SEQ ID NO: 225 - protein, 122 aa, Artificial Sequence
  Amino acid sequence of the variable region of the heavy chain of anti-hTfR antibody No.4
EVQLQESGAELVRPGTSVRVFCKASGYAFTNYLIEWVKQRPGQGLEWIGLINPGSGGIIYNEKFTDRATLTADKSSSTAYMQLSSLTSDDSAVYFCARSNYYGTTYWHFDVWGAGTTVTVSS

SEQ ID NO: 226 - protein, 105 aa, Artificial Sequence
  Amino acid sequence of the variable region of the light chain of anti-hTfR antibody No.5
DIVMTQTPAIMSASPGEKVTMTCSASSSISSIHWYQQKPGTSPKRWIYDTSTLASGVPVRFSGSGSGTSYSLTISSMEAEDAATYYCHQRSSYPTFGGGTKLEIK

SEQ ID NO: 227 - protein, 118 aa, Artificial Sequence
  Amino acid sequence of the variable region of the heavy chain of anti-hTfR antibody No.5
EVQLQESGPELVKPGASVKMSCKASGYTFTNFVIHWVKQRPGQGLEWIGFFNPHKNGAEYNEKFQVKATLTSDKSSTTAYMELNSLTSEDSAVYYCARSFYYYSMDYWGQGTSVTVSS

SEQ ID NO: 228 - protein, 107 aa, Artificial Sequence
  Amino acid sequence of the variable region of the light chain of anti-hTfR antibody No.6
DIVLTQTPSSLSASLGERVSLTCRASQEISGYLSWLQQKPDGTIKRLIYAASTLDSGVPKRFSGSRSGSDYSLTISSLESEDFADYYCLQYSSYPRTFGGGTKLEIK

SEQ ID NO: 229 - protein, 112 aa, Artificial Sequence
  Amino acid sequence of the variable region of the heavy chain of anti-hTfR antibody No.6
EVQLQESGPGLVAPSQSLSITCSVSGFSLSTYGVYWVRQPPGKGLEWLGIIWGDGSTNYHSALISRLTISKDNSKSQVFLKLNSLQTADTATYYCAKPDDVWGAGTTVTVSS

SEQ ID NO: 230 - protein, 106 aa, Artificial Sequence
  Amino acid sequence of the variable region of the light chain of anti-hTfR antibody No.7
DIVLTQSPVIMSASLGEEITLTCSASSSVNYIHWYQQKSGTSPKVLIYQTSNLASGVPSRFSGSRSGTFYSLKISSVEAEDAADYYCHQWSSYPWTFGGGTKLEIK

SEQ ID NO: 231 - protein, 120 aa, Artificial Sequence
  Amino acid sequence of the variable region of the heavy chain of anti-hTfR antibody No.7
EVQLQESGGALVKPGGSLKVSCEASGITFRNYFMSWVRQTPEKRLEWVATISSAGGYTYYADSVKGRFTISRDNAGNTLYLQMSSLRSEDTAMYFCARQEVPYPYAMDYWGQGTSVIVSS

SEQ ID NO: 232 - protein, 106 aa, Artificial Sequence
  Amino acid sequence of the variable region of the light chain of anti-hTfR antibody No.8
DIVLTQSPAIMSASLGEEITLTCSASSSVSYMHWYQQKSGTSPKVLIYGTSNLASEVPSRFSGSGSGTFYSLTISSVEAEDAADYYCHQWSSYPWTFGGGTKLEIK

SEQ ID NO: 233 - protein, 112 aa, Artificial Sequence
  Amino acid sequence of the variable region of the heavy chain of anti-hTfR antibody No.8
EVQLQESGPGLVAPSQSLSITCTVSGFSLTTYGVSWIRQPPGKGLEWLGIIWGDGSTNYRSALISRLSISKDNSKNQVFLKLNSLQTDDTATYYCAKPDDYWGQGTSVTVSS

SEQ ID NO: 234 - protein, 106 aa, Artificial Sequence
  Amino acid sequence of the variable region of the light chain of anti-hTfR antibody No.9
DIVLTQSPALMSASPGETVTMTCSASSSVSLMFWYQQKPRSSPKPWIYFTSYRASGVPIRFSGSGSGTSFSLTISNLEAEDAATYYCQQWTSDPPTFGSGTKLEIE

SEQ ID NO: 235 - protein, 117 aa, Artificial Sequence
  Amino acid sequence of the variable region of the heavy chain of anti-hTfR antibody No.9
EVQLQESGPELKKPGETVKISCKASGYTFTNYGVSWVKQAPGKDLKWMGWIYTFTGEATYIDDFRGRFAFSLETSANTAYLQINNLKNEDTATYFCSRRNGAWFEDWGQGTLVTVSA

SEQ ID NO: 236 - protein, 107 aa, Artificial Sequence
  Amino acid sequence of the variable region of the light chain of anti-hTfR antibody No.10
DIVMTQTPSSLSASLGERVSLTCRPSQEISGYLSWLQQKPDGTIKRLIYAASTLDSGVPKRFSGSRSGSDYSLTISSLESEDFADYYCLQYASYPRTFGGGTKLEIK

SEQ ID NO: 237 - protein, 120 aa, Artificial Sequence
  Amino acid sequence of the variable region of the heavy chain of anti-hTfR antibody No.10
EVQLQESGGGLVKPGGSLKLSCEASGITFRNYAMSWVRQTPEKRLEWVATISSYGGYTYYADSVKGRFTVSRDNAGNTLYLQMSSLRSEDTAMYHCARQEVPYPYPMDNWGQGTSVIVSS

SEQ ID NO: 238 - protein, 107 aa, Artificial Sequence
  Amino acid sequence of the variable region of the light chain of anti-hTfR antibody No.11
DIVLTQSPATLSVTPGDRVSLSCRASQSIRNYLHWYQQKSHESPRLLIKYASQSISGIPSRFSGSGSGTDFTLSINSVETEDFGMYFCQQTNSWPYTFGGGTKLEIK

SEQ ID NO: 239 - protein, 118 aa, Artificial Sequence
  Amino acid sequence of the variable region of the heavy chain of anti-hTfR antibody No.11
EVQLQESGAELVRPGSSVKISCKASGYAFSIYWINWLKQRPGQGLEWIGQIYPGNGDTNYNGKFKGKATLTADKSSNTVYMRLSSLTSEDSAVYFCGRWGDDYAMDFWGQGTSVTVSS

SEQ ID NO: 240 - protein, 107 aa, Artificial Sequence
  Amino acid sequence of the variable region of the light chain of anti-hTfR antibody No.12
DIVLTQSHKFMSTVIGDRVSITCKASHDVKTAVAWYQQTPGQSPKLLTYWSSTRHTGVPDRFTGSGSGTDYTLTISSVQAEDLALYYCQQHFSTPLTFGAGTKLELK

SEQ ID NO: 241 - protein, 119 aa, Artificial Sequence
  Amino acid sequence of the variable region of the heavy chain of anti-hTfR antibody No.12
EVQLQESGAELARPGTSVKVSCKAAGYVFINYLIEWVKQRPGQGLEWIGVIHSGSGGTNYNDNFKDKATLTRDVSSSTAYMQLSSLTSDDSAVYFCARRNFGNYYFDYWGQGTTLTVSS

SEQ ID NO: 242 - protein, 107 aa, Artificial Sequence
  Amino acid sequence of the variable region of the light chain of anti-hTfR antibody No.13
DIVITQTPATLSVTPGDRVSLSCRASQSIRNYLHWYQQKSHESPRLLIKYASQSISGIPSRFSGSGSGTDFTLTINSVETEDFGMYFCQQTNSWPYTFGGGTKLEIK

SEQ ID NO: 243 - protein, 118 aa, Artificial Sequence; identical to SEQ ID NO: 239
  Amino acid sequence of the variable region of the heavy chain of anti-hTfR antibody No.13

SEQ ID NO: 244 - protein, 106 aa, Artificial Sequence
  Amino acid sequence of the variable region of the light chain of anti-hTfR antibody No.14
DIVLTQTPVIMSAYPGEKVTLTCSASSNINSIHWYQQKPGTSPKRWIYDTSNLASGVPARFSGSGSGTSYSLTISSMEAEDAASYYCHQRSGYPFTFGSGTKLEIK

SEQ ID NO: 245 - protein, 118 aa, Artificial Sequence
  Amino acid sequence of the variable region of the heavy chain of anti-hTfR antibody No.14
EVQLQESGPELLKPGASVKMSCKASGYAFTGYVIHWVKQKPGQGLEWIGFLNPHKDDSEYNEKFRGKATLTSDKSSSTAYMDLSSLTSEDSAVYYCARGYYYYSMDYWGQGTSVTVSS

SEQ ID NO: 246 - protein, 525 aa, Homo sapiens
SETQANSTTDALNVLLIIVDDLRPSLGCYGDKLVRSPNIDQLASHSLLFQNAFAQQAVCAPSRVSFLTGRRPDTTRLYDFNSYWRVHAGNFSTIPQYFKENGYVTMSVGKVFHPGISSNHTDDSPYSWSFPPYHPSSEKYENTKTCRGPDGELHANLLCPVDVLDVPEGTLPDKQSTEQAIQLLEKMKTSASPFFLAVGYHKPHIPFRYPKEFQKLYPLENITLAPDPEVPDGLPPVAYNPWMDIRQREDVQALNISVPYGPIPVDFQRKIRQSYFASVSYLDTQVGRLLSALDDLQLANSTIIAFTSDHGWALGEHGEWAKYSNFDVATHVPLIFYVPGRTASLPEAGEKLFPYLDPFDSASQLMEPGRQSMDLVELVSLFPTLAGLAGLQVPPRCPVPSFHVELCREGKNLLKHFRFRDLEEDPYLPGNPRELIAYSQYPRPSDIPQWNSDKPSLKDIKIMGYSIRTIDYRYTVWVGFNPDEFLANFSDIHAGELYFVDSDPLQDHNMYNDSQGGDLFQLLMP

SEQ ID NO: 247 - protein, 973 aa, Artificial Sequence
  Amino acid sequence of the fusion protein of heavy chain of anti-hTfR antibody No.1 (humanized 6) and hI2S
EVQLVESGGGLVQPGGSLRLSCAASGLTFSNYGMSWVRQAPGKGLELVANINTNGGSTYYPDSVKGRFTISRDNAKNSLYLQMNSLRAEDTAVYYCTNNRYDEDYWGQGTLVTVSSASTKGPSVFPLAPSSKSTSGGTAALGCLVKDYFPEPVTVSWNSGALTSGVHTFPAVLQSSGLYSLSSVVTVPSSSLGTQTYICNVNHKPSNTKVDKKVEPKSCDKTHTCPPCPAPELLGGPSVFLFPPKPKDTLMISRTPEVTCVVVDVSHEDPEVKFNWYVDGVEVHNAKTKPREEQYNSTYRVVSVLTVLHQDWLNGKEYKCKVSNKALPAPIEKTISKAKGQPREPQVYTLPPSRDELTKNQVSLTCLVKGFYPSDIAVEWESNGQPENNYKTTPPVLDSDGSFFLYSKLTVDKSRWQQGNVFSCSVMHEALHNHYTQKSLSLSPGKGSSETQANSTTDALNVLLIIVDDLRPSLGCYGDKLVRSPNIDQLASHSLLFQNAFAQQAVCAPSRVSFLTGRRPDTTRLYDFNSYWRVHAGNFSTIPQYFKENGYVTMSVGKVFHPGISSNHTDDSPYSWSFPPYHPSSEKYENTKTCRGPDGELHANLLCPVDVLDVPEGTLPDKQSTEQAIQLLEKMKTSASPFFLAVGYHKPHIPFRYPKEFQKLYPLENITLAPDPEVPDGLPPVAYNPWMDIRQREDVQALNISVPYGPIPVDFQRKIRQSYFASVSYLDTQVGRLLSALDDLQLANSTIIAFTSDHGWALGEHGEWAKYSNFDVATHVPLIFYVPGRTASLPEAGEKLFPYLDPFDSASQLMEPGRQSMDLVELVSLFPTLAGLAGLQVPPRCPVPSFHVELCREGKNLLKHFRFRDLEEDPYLPGNPRELIAYSQYPRPSDIPQWNSDKPSLKDIKIMGYSIRTIDYRYTVWVGFNPDEFLANFSDIHAGELYFVDSDPLQDHNMYNDSQGGDLFQLLMP

SEQ ID NO: 248 - DNA, 3002 bp, Artificial Sequence
  Nucleotide sequence encoding the amino acid sequence of fusion protein of heavy chain of anti-hTfR antibody No.1 (humanized 6) and hI2S, synthetic sequence
acgcgtgccgccaccatgggctggagctggattctgctgttcctcctgagcgtgacagcaggagtgcacagcgaagtgcagctggtcgaatcagggggggggctggtgcagcctggaggcagcctgagactgtcctgcgccgcttctggcttgacctttagcaactacgggatgtcctgggtgcggcaggctcctggcaagggactggagttggtggccaacatcaataccaacggcggaagtacatactatcccgattcagtgaagggccggttcaccatcagcagggacaacgccaagaacagcctgtatctgcagatgaactctctgagggccgaggatacagccgtgtactattgcactaacaaccggtacgacgaggactattggggccagggcaccctggtgacagtgtctagcgcctctaccaagggcccaagcgtgtttcctctggctccatcctctaaatccacctctggcggcacagccgctctgggctgtctggtgaaggattacttcccagagcccgtgacagtgtcttggaacagcggcgccctgacctccggcgtgcacacatttcctgctgtgctgcagagctccggcctgtacagcctgtctagcgtggtgaccgtgccatcctctagcctgggcacccagacatatatctgcaacgtgaatcacaagcccagcaatacaaaggtggataagaaggtggagccaaagtcctgtgacaagacccacacatgccccccttgtcctgctccagagctgctgggaggaccaagcgtgttcctgtttccacccaagcccaaggataccctgatgatctctcggaccccagaggtgacatgcgtggtggtggatgtgagccacgaggaccccgaggtgaagttcaactggtatgtggacggcgtggaggtgcacaatgctaagaccaagcccagggaggagcagtacaactccacctatagagtggtgtctgtgctgacagtgctgcaccaggattggctgaacggcaaggagtataagtgcaaggtgtccaataaggccctgcccgctcctatcgagaagaccatctctaaggccaagggccagcccagagagcctcaggtgtacacactgcctccatcccgggatgagctgaccaagaaccaggtgtctctgacatgtctggtcaagggcttctatccctctgacatcgccgtggagtgggagagcaatggccagcctgagaacaattacaagaccacaccccctgtgctggattccgacggctctttctttctgtatagcaagctgaccgtggacaagtcccggtggcagcagggcaacgtgttcagctgttccgtgatgcacgaagctctgcataatcactatactcagaaatccctgtcactgtcacctggtaaaggatcttccgaaacgcaggccaactcgaccacagatgctctgaacgttcttctcatcatcgtggatgacctgcgcccctccctgggctgttatggggataagctggtgaggtccccaaatattgaccaactggcatcccacagcctcctcttccagaatgcctttgcgcagcaagcagtgtgcgccccgagccgcgtttctttcctcactggcaggagacctgacaccacccgcctgtacgacttcaactcctactggagggtgcacgctggaaacttctccaccatcccccagtacttcaaggagaatggctatgtgaccatgtcggtgggaaaagtctttcaccctgggatatcttctaaccataccgatgattctccgtatagctggtcttttccaccttatcatccttcctctgagaagtatgaaaacactaagacatgtcgagggccagatggagaactccatgccaacctgctttgccctgtggatgtgctggatgttcccgagggcaccttgcctgacaaacagagcactgagcaagccatacagttgttggaaaagatgaaaacgtcagccagtcctttcttcctggccgttgggtatcataagccacacatccccttcagataccccaaggaatttcagaagttgtatcccttggagaacatcaccctggcccccgatcccgaggtccctgatggcctaccccctgtggcctacaacccctggatggacatcaggcaacgggaagacgtccaagccttaaacatcagtgtgccgtatggtccaattcctgtggactttcagcggaaaatccgccagagctactttgcctctgtgtcatatttggatacacaggtcggccgcctcttgagtgctttggacgatcttcagctggccaacagcaccatcattgcatttacctcggatcatgggtgggctctaggtgaacatggagaatgggccaaatacagcaattttgatgttgctacccatgttcccctgatattctatgttcctggaaggacggcttcacttccggaggcaggcgagaagcttttcccttacctcgacccttttgattccgcctcacagttgatggagccaggcaggcaatccatggaccttgtggaacttgtgtctctttttcccacgctggctggacttgcaggactgcaggttccacctcgctgccccgttccttcatttcacgttgagctgtgcagagaaggcaagaaccttctgaagcattttcgattccgtgacttggaagaagatccgtacctccctggtaatccccgtgaactgattgcctatagccagtatccccggccttcagacatccctcagtggaattctgacaagccgagtttaaaagatataaagatcatgggctattccatacgcaccatagactataggtatactgtgtgggttggcttcaatcctgatgaatttctagctaacttttctgacatccatgcaggggaactgtattttgtggattctgacccattgcaggatcacaatatgtataatgattcccaaggtggagaccttttccagttgttgatgccttaagcggccgc

SEQ ID NO: 249 - protein, 980 aa, Artificial Sequence
  Amino acid sequence of the fusion protein of heavy chain of anti-hTfR antibody No.2 (humanized 6) and hI2S
QVQLVQSGAEVKKPGASVKVSCKASGYTFTDYVMHWVRQAPGQGLEWIGVISTYYGHGSYNQRFKGRATMTVDKSISTAYMELVRLRSDDTAVYYCVRGGYGSSSLAGNFDVWGQGTTVTVSSASTKGPSVFPLAPSSKSTSGGTAALGCLVKDYFPEPVTVSWNSGALTSGVHTFPAVLQSSGLYSLSSVVTVPSSSLGTQTYICNVNHKPSNTKVDKKVEPKSCDKTHTCPPCPAPELLGGPSVFLFPPKPKDTLMISRTPEVTCVVVDVSHEDPEVKFNWYVDGVEVHNAKTKPREEQYNSTYRVVSVLTVLHQDWLNGKEYKCKVSNKALPAPIEKTISKAKGQPREPQVYTLPPSRDELTKNQVSLTCLVKGFYPSDIAVEWESNGQPENNYKTTPPVLDSDGSFFLYSKLTVDKSRWQQGNVFSCSVMHEALHNHYTQKSLSLSPGKGSSETQANSTTDALNVLLIIVDDLRPSLGCYGDKLVRSPNIDQLASHSLLFQNAFAQQAVCAPSRVSFLTGRRPDTTRLYDFNSYWRVHAGNFSTIPQYFKENGYVTMSVGKVFHPGISSNHTDDSPYSWSFPPYHPSSEKYENTKTCRGPDGELHANLLCPVDVLDVPEGTLPDKQSTEQAIQLLEKMKTSASPFFLAVGYHKPHIPFRYPKEFQKLYPLENITLAPDPEVPDGLPPVAYNPWMDIRQREDVQALNISVPYGPIPVDFQRKIRQSYFASVSYLDTQVGRLLSALDDLQLANSTIIAFTSDHGWALGEHGEWAKYSNFDVATHVPLIFYVPGRTASLPEAGEKLFPYLDPFDSASQLMEPGRQSMDLVELVSLFPTLAGLAGLQVPPRCPVPSFHVELCREGKNLLKHFRFRDLEEDPYLPGNPRELIAYSQYPRPSDIPQWNSDKPSLKDIKIMGYSIRTIDYRYTVWVGFNPDEFLANFSDIHAGELYFVDSDPLQDHNMYNDSQGGDLFQLLMP

SEQ ID NO: 250 - DNA, 3023 bp, Artificial Sequence
  Nucleotide sequence encoding the amino acid sequence of fusion protein of heavy chain of anti-hTfR antibody No.2 (humanized 6) and hI2S, synthetic sequence
acgcgtgccgccaccatgggctggagctggattctgctgttcctcctgagcgtgacagcaggagtgcacagccaggtgcagctggtccagtcaggagccgaagtgaaaaagcccggagcctcagtcaaagtgtcttgtaaagcatcaggttatacatttacagactacgtcatgcactgggtgaggcaggcacctggacagggtctggaatggatcggcgtgatctccacttactatggccatggaagctacaaccagagattcaagggcagggcgacaatgactgtagacaaatcaatttccactgcttatatggagctggtaaggctgcggtccgacgataccgctgtgtactattgcgtacgaggaggatacggctccagctctctggctggtaatttcgatgtgtgggggcagggtaccacagtcaccgtgagttcagcaagcacaaagggcccatctgtgtttccactggccccctccagcaaaagcacctctgggggtacagccgctctgggatgtctggtgaaggattatttcccagagccagtcaccgtgtcctggaacagcggagccctgacatctggagtccacacttttccagctgtgctgcagtctagtgggctgtactccctgtcatccgtggtcactgtccccagctctagtctgggtacccagacatatatctgcaacgtgaatcacaagccatctaataccaaagtcgacaagaaagtggaacccaagtcctgtgataaaactcatacctgccccccttgtcctgcaccagagctgctgggaggaccatccgtgttcctgtttccacccaagcctaaagacaccctgatgattagccgaactcccgaagtcacctgcgtggtcgtggacgtgtctcacgaggaccctgaagtcaagtttaactggtacgtggatggcgtcgaggtgcataatgctaagacaaaaccccgagaggaacagtacaacagtacatatcgtgtcgtgtcagtgctgaccgtcctgcatcaggactggctgaacgggaaggaatataagtgcaaagtgtccaataaggcactgcccgcccctatcgagaaaaccattagcaaggccaaaggacagcctagggaaccacaggtgtacacactgcctccatcccgggacgagctgactaagaaccaggtcagcctgacctgtctggtgaaaggcttctatccttcagatatcgctgtggagtgggaaagtaatggacagccagagaacaattacaagactaccccccctgtgctggactctgatgggagtttctttctgtattctaagctgaccgtggataaaagtcggtggcagcagggtaatgtctttagttgttcagtgatgcacgaagcactgcacaaccactacacccagaaatcactgtcactgtcaccagggaaaggatcttccgaaacgcaggccaactcgaccacagatgctctgaacgttcttctcatcatcgtggatgacctgcgcccctccctgggctgttatggggataagctggtgaggtccccaaatattgaccaactggcatcccacagcctcctcttccagaatgcctttgcgcagcaagcagtgtgcgccccgagccgcgtttctttcctcactggcaggagacctgacaccacccgcctgtacgacttcaactcctactggagggtgcacgctggaaacttctccaccatcccccagtacttcaaggagaatggctatgtgaccatgtcggtgggaaaagtctttcaccctgggatatcttctaaccataccgatgattctccgtatagctggtcttttccaccttatcatccttcctctgagaagtatgaaaacactaagacatgtcgagggccagatggagaactccatgccaacctgctttgccctgtggatgtgctggatgttcccgagggcaccttgcctgacaaacagagcactgagcaagccatacagttgttggaaaagatgaaaacgtcagccagtcctttcttcctggccgttgggtatcataagccacacatccccttcagataccccaaggaatttcagaagttgtatcccttggagaacatcaccctggcccccgatcccgaggtccctgatggcctaccccctgtggcctacaacccctggatggacatcaggcaacgggaagacgtccaagccttaaacatcagtgtgccgtatggtccaattcctgtggactttcagcggaaaatccgccagagctactttgcctctgtgtcatatttggatacacaggtcggccgcctcttgagtgctttggacgatcttcagctggccaacagcaccatcattgcatttacctcggatcatgggtgggctctaggtgaacatggagaatgggccaaatacagcaattttgatgttgctacccatgttcccctgatattctatgttcctggaaggacggcttcacttccggaggcaggcgagaagcttttcccttacctcgacccttttgattccgcctcacagttgatggagccaggcaggcaatccatggaccttgtggaacttgtgtctctttttcccacgctggctggacttgcaggactgcaggttccacctcgctgccccgttccttcatttcacgttgagctgtgcagagaaggcaagaaccttctgaagcattttcgattccgtgacttggaagaagatccgtacctccctggtaatccccgtgaactgattgcctatagccagtatccccggccttcagacatccctcagtggaattctgacaagccgagtttaaaagatataaagatcatgggctattccatacgcaccatagactataggtatactgtgtgggttggcttcaatcctgatgaatttctagctaacttttctgacatccatgcaggggaactgtattttgtggattctgacccattgcaggatcacaatatgtataatgattcccaaggtggagaccttttccagttgttgatgccttaagcggccgc

SEQ ID NO: 251 - protein, 975 aa, Artificial Sequence
  Amino acid sequence of fusion protein of heavy chain of anti-hTfR antibody No.3 (humanized 2) and hI2S, synthetic sequence
EVQLVQSGAEVKKPGESLKISCKGSGYSFTNYWLGWVRQMPGKGLEWMGDIYPGGDYPTYSEKFKVQVTISADKSISTAYLQWSSLKASDTAMYYCARSGNYDEVAYWGQGTLVTVSSASTKGPSVFPLAPSSKSTSGGTAALGCLVKDYFPEPVTVSWNSGALTSGVHTFPAVLQSSGLYSLSSVVTVPSSSLGTQTYICNVNHKPSNTKVDKKVEPKSCDKTHTCPPCPAPELLGGPSVFLFPPKPKDTLMISRTPEVTCVVVDVSHEDPEVKFNWYVDGVEVHNAKTKPREEQYNSTYRVVSVLTVLHQDWLNGKEYKCKVSNKALPAPIEKTISKAKGQPREPQVYTLPPSRDELTKNQVSLTCLVKGFYPSDIAVEWESNGQPENNYKTTPPVLDSDGSFFLYSKLTVDKSRWQQGNVFSCSVMHEALHNHYTQKSLSLSPGKGSSETQANSTTDALNVLLIIVDDLRPSLGCYGDKLVRSPNIDQLASHSLLFQNAFAQQAVCAPSRVSFLTGRRPDTTRLYDFNSYWRVHAGNFSTIPQYFKENGYVTMSVGKVFHPGISSNHTDDSPYSWSFPPYHPSSEKYENTKTCRGPDGELHANLLCPVDVLDVPEGTLPDKQSTEQAIQLLEKMKTSASPFFLAVGYHKPHIPFRYPKEFQKLYPLENITLAPDPEVPDGLPPVAYNPWMDIRQREDVQALNISVPYGPIPVDFQRKIRQSYFASVSYLDTQVGRLLSALDDLQLANSTIIAFTSDHGWALGEHGEWAKYSNFDVATHVPLIFYVPGRTASLPEAGEKLFPYLDPFDSASQLMEPGRQSMDLVELVSLFPTLAGLAGLQVPPRCPVPSFHVELCREGKNLLKHFRFRDLEEDPYLPGNPRELIAYSQYPRPSDIPQWNSDKPSLKDIKIMGYSIRTIDYRYTVWVGFNPDEFLANFSDIHAGELYFVDSDPLQDHNMYNDSQGGDLFQLLMP

SEQ ID NO: 252 - DNA, 3011 bp, Artificial Sequence
  Nucleotide sequence encoding the amino acid sequence of fusion protein of heavy chain of anti-hTfR antibody No.3 (humanized 2) and hI2S, synthetic sequence
acgcgtgccgccaccatgggctggagctggattctgctgttcctcctgagcgtgacagcaggagtgcacagcgaggtgcaactagtgcagtctggagcagaggtgaaaaagcccggggagtctctgaagatttcctgtaagggttctggatacagctttaccaactactggctgggatgggtgcgccagatgcccgggaaaggcctggagtggatgggggacatctaccccggcggagactaccctacatacagcgagaagttcaaggtccaggtcaccatctcagccgacaagtccatcagcaccgcctacctgcagtggagcagcctgaaggcctcggacaccgccatgtattactgtgcgagatcaggcaattacgacgaagtggcctactggggccaaggaaccctggtcaccgtctcctcagctagcaccaagggcccatcggtcttccccctggcaccctcctccaagagcacctctgggggcacagcggccctgggctgcctggtcaaggactacttccccgaaccggtgacggtgtcgtggaactcaggcgccctgaccagcggcgtgcacaccttcccggctgtcctacagtcctcaggactctactccctcagcagcgtggtgaccgtgccctccagcagcttgggcacccagacctacatctgcaacgtgaatcacaagcccagcaacaccaaggtggacaagaaagttgagcccaaatcttgtgacaaaactcacacgtgcccaccgtgcccagcacctgaactcctgggaggtccgtcagtcttcctcttccccccaaaacccaaggacaccctcatgatctcccggacccctgaggtcacatgcgtggtggtggacgtgagccacgaagaccctgaggtcaagttcaactggtacgtggacggcgtggaggtgcataatgccaagacaaagccgcgggaggagcagtacaacagcacgtaccgggtggtcagcgtcctcaccgtcctgcaccaggactggctgaatggcaaggagtacaagtgcaaggtctccaacaaagccctcccagcccccatcgagaaaaccatctccaaagccaaagggcagccccgagaaccacaggtgtacaccctgcccccatcccgggatgagctgaccaagaaccaggtcagcctgacctgcctggtcaaaggcttctatcccagcgacatcgccgtggagtgggagagcaatgggcagccggagaacaactacaagaccacgcctcccgtgctggactccgacggctccttcttcctctacagcaagctcaccgtggacaagagcaggtggcagcaggggaacgtcttctcatgctccgtgatgcatgaggctctgcacaaccactacacgcagaagagcctctccctgtctccgggtaaaggatcttccgaaacgcaggccaactcgaccacagatgctctgaacgttcttctcatcatcgtggatgacctgcgcccctccctgggctgttatggggataagctggtgaggtccccaaatattgaccaactggcatcccacagcctcctcttccagaatgcctttgcgcagcaagcagtgtgcgccccgagccgcgtttctttcctcactggcaggagacctgacaccacccgcctgtacgacttcaactcctactggagggtgcacgctggaaacttctccaccatcccccagtacttcaaggagaatggctatgtgaccatgtcggtgggaaaagtctttcaccctgggatatcttctaaccataccgatgattctccgtatagctggtcttttccaccttatcatccttcctctgagaagtatgaaaacactaagacatgtcgagggccagatggagaactccatgccaacctgctttgccctgtggatgtgctggatgttcccgagggcaccttgcctgacaaacagagcactgagcaagccatacagttgttggaaaagatgaaaacgtcagccagtcctttcttcctggccgttgggtatcataagccacacatccccttcagataccccaaggaatttcagaagttgtatcccttggagaacatcaccctggcccccgatcccgaggtccctgatggcctaccccctgtggcctacaacccctggatggacatcaggcaacgggaagacgtccaagccttaaacatcagtgtgccgtatggtccaattcctgtggactttcagcggaaaatccgccagagctactttgcctctgtgtcatatttggatacacaggtcggccgcctcttgagtgctttggacgatcttcagctggccaacagcaccatcattgcatttacctcggatcatgggtgggctctaggtgaacatggagaatgggccaaatacagcaattttgatgttgctacccatgttcccctgatattctatgttcctggaaggacggcttcacttccggaggcaggcgagaagcttttcccttacctcgacccttttgattccgcctcacagttgatggagccaggcaggcaatccatggaccttgtggaacttgtgtctctttttcccacgctggctggacttgcaggactgcaggttccacctcgctgccccgttccttcatttcacgttgagctgtgcagagaaggcaagaaccttctgaagcattttcgattccgtgacttggaagaagatccgtacctccctggtaatccccgtgaactgattgcctatagccagtatccccggccttcagacatccctcagtggaattctgacaagccgagtttaaaagatataaagatcatgggctattccatacgcaccatagactataggtatactgtgtgggttggcttcaatcctgatgaatttctagctaacttttctgacatccatgcaggggaactgtattttgtggattctgacccattgcaggatcacaatatgtataatgattcccaaggtggagaccttttccagttgttgatgccttaataagcggccgc

SEQ ID NO: 253 - DNA, 4460 bp, Artificial Sequence
  Nucleotide sequence of the DNA formed of a cDNA encoding chimeric hTfR and a loxP-flanked neomycin resistance gene placed on the cDNA's 3' side, synthetic sequence
gtttatcctcccttgtagcagctgagaatgatggatcaagccagatcagcattctctaacttgtttggtggggaaccattgtcatacacccggtttagccttgctcggcaagtagatggagataacagtcatgtggagatgaaactggctgcagatgaagaagaaaatgccgacaataacatgaaggctagtgtcagaaaacccaagaggtttaatggaagactctgctttgcagctattgcactagtcattttcttcttgattggattcatgagtggctacctgggctattgtaaaggggtagaaccaaaaactgagtgtgagagactggcaggaaccgagtctccagtgagggaggagccaggagaggacttccctgcagcacgtcgcttatattgggatgacctgaagagaaagttgtcggagaaactggacagcacagacttcaccggcaccatcaagctgctgaatgaaaattcatatgtccctcgtgaggctggatctcaaaaagatgaaaatcttgcgttgtatgttgaaaatcaatttcgtgaatttaaactcagcaaagtctggcgtgatcaacattttgttaagattcaggtcaaagacagcgctcaaaactcggtgatcatagttgataagaacggtagacttgtttacctggtggagaatcctgggggttatgtggcgtatagtaaggctgcaacagttactggtaaactggtccatgctaattttggtactaaaaaagattttgaggatttatacactcctgtgaatggatctatagtgattgtcagagcagggaaaatcacctttgcagaaaaggttgcaaatgctgaaagcttaaatgcaattggtgtgttgatatacatggaccagactaaatttcccattgttaacgcagaactttcattctttggacatgctcatctggggacaggtgacccttacacacctggattcccttccttcaatcacactcagtttccaccatctcggtcatcaggattgcctaatatacctgtccagacaatctccagagctgctgcagaaaagctgtttgggaatatggaaggagactgtccctctgactggaaaacagactctacatgtaggatggtaacctcagaaagcaagaatgtgaagctcactgtgagcaatgtgctgaaagagataaaaattcttaacatctttggagttattaaaggctttgtagaaccagatcactatgttgtagttggggcccagagagatgcatggggccctggagctgcaaaatccggtgtaggcacagctctcctattgaaacttgcccagatgttctcagatatggtcttaaaagatgggtttcagcccagcagaagcattatctttgccagttggagtgctggagactttggatcggttggtgccactgaatggctagagggatacctttcgtccctgcatttaaaggctttcacttatattaatctggataaagcggttcttggtaccagcaacttcaaggtttctgccagcccactgttgtatacgcttattgagaaaacaatgcaaaatgtgaagcatccggttactgggcaatttctatatcaggacagcaactgggccagcaaagttgagaaactcactttagacaatgctgctttccctttccttgcatattctggaatcccagcagtttctttctgtttttgcgaggacacagattatccttatttgggtaccaccatggacacctataaggaactgattgagaggattcctgagttgaacaaagtggcacgagcagctgcagaggtcgctggtcagttcgtgattaaactaacccatgatgttgaattgaacctggactatgagaggtacaacagccaactgctttcatttgtgagggatctgaaccaatacagagcagacataaaggaaatgggcctgagtttacagtggctgtattctgctcgtggagacttcttccgtgctacttccagactaacaacagatttcgggaatgctgagaaaacagacagatttgtcatgaagaaactcaatgatcgtgtcatgagagtggagtatcacttcctctctccctacgtatctccaaaagagtctcctttccgacatgtcttctggggctccggctctcacacgctgccagctttactggagaacttgaaactgcgtaaacaaaataacggtgcttttaatgaaacgctgttcagaaaccagttggctctagctacttggactattcagggagctgcaaatgccctctctggtgacgtttgggacattgacaatgagttttaacgtggctcgctgatcagcctcgactgtgccttctagttgccagccatctgttgtttgcccctcccccgtgccttccttgaccctggaaggtgccactcccactgtcctttcctaataaaatgaggaaattgcatcgcattgtctgagtaggtgtcattctattctggggggtggggtggggcaggacagcaagggggaggattgggaagacaatagcaggcatgctggggatgcggtgggctctatggcttctgaggcggaaagaaccagctggggctcgatcctctagttaagcttcccagcggccgctatcgaattccgatcatattcaataacccttaatataacttcgtataatgtatgctatacgaagttattaggtctgaagaggagtttacgtccagccaagctaattctaccgggtaggggaggcgcttttcccaaggcagtctggagcatgcgctttagcagccccgctgggcacttggcgctacacaagtggcctctggcctcgcacacattccacatccaccggtaggcgccaaccggctccgttctttggtggccccttcgcgccaccttctactcctcccctagtcaggaagttcccccccgccccgcagctcgcgtcgtgcaggacgtgacaaatggaagtagcacgtctcactagtctcgtgcagatggacagcaccgctgagcaatggaagcgggtaggcctttggggcagcggccaatagcagctttgctccttcgctttctgggctcagaggctgggaaggggtgggtccgggggcgggctcaggggcgggctcaggggcggggcgggcgcccgaaggtcctccggaggcccggcattctgcacgcttcaaaagcgcacgtctgccgcgctgttctcctcttcctcatctccgggcctttcgacctgcagccaatatgggatcggccattgaacaagatggattgcacgcaggttctccggccgcttgggtggagaggctattcggctatgactgggcacaacagacaatcggctgctctgatgccgccgtgttccggctgtcagcgcaggggcgcccggttctttttgtcaagaccgacctgtccggtgccctgaatgaactgcaggacgaggcagcgcggctatcgtggctggccacgacgggcgttccttgcgcagctgtgctcgacgttgtcactgaagcgggaagggactggctgctattgggcgaagtgccggggcaggatctcctgtcatctcaccttgctcctgccgagaaagtatccatcatggctgatgcaatgcggcggctgcatacgcttgatccggctacctgcccattcgaccaccaagcgaaacatcgcatcgagcgagcacgtactcggatggaagccggtcttgtcgatcaggatgatctggacgaagagcatcaggggctcgcgccagccgaactgttcgccaggctcaaggcgcgcatgcccgacggcgaggatctcgtcgtgacccatggcgatgcctgcttgccgaatatcatggtggaaaatggccgcttttctggattcatcgactgtggccggctgggtgtggcggaccgctatcaggacatagcgttggctacccgtgatattgctgaagagcttggcggcgaatgggctgaccgcttcctcgtgctttacggtatcgccgctcccgattcgcagcgcatcgccttctatcgccttcttgacgagttcttctgaggggatccgctgtaagtctgcagaaattgatgatctattaaacaataaagatgtccactaaaatggaagtttttcctgtcatactttgttaagaagggtgagaacagagtacctacattttgaatggaaggattggagctacgggggtgggggtggggtgggattagataaatgcctgctctttactgaaggctctttactattgctttatgataatgtttcatagttggatatcataatttaaacaagcaaaaccaaattaagggccagctcattcctcccactcatgatctatagatccctcgatcgagatccggaacccttaatataacttcgtataatgtatgctatacgaagttattaggtccctcgaagaggttcactagttctagagcatttaaatacgtgctagc

SEQ ID NO: 254 - DNA, 5003 bp, Artificial Sequence
  Nucleotide sequence of the 5'-arm of targeting vector
aaagacattcccagggtccctaagggctccatctgggagcgcgctatctgtagtcctgttgtggtttaagataccactctctttgttatttgtaaatttaccacaggctgggcagtaaagtacagataggaagaaaagagtgtgaacgtttgcagttttaacagaactccttttatttgctatgcattgcaacaaccctctaaaagcaataatggcgataaacatgcaagttaatctacaactttatcaccctagtaaatcattggttcctatttcccttccataggctgaacatagtgagcactggtagctctttgcttggcttaagcgctgcttgttaaaatctaaaaaaaaaaaaaaaaaagatttgcagttttgctttaaagtttttcctttaaagcatctctgagctgcaaaaactcgtctttaggatatggttttggcggagacctaagcctgcaagtaggaatattttaaagagtaaaggctgatactttcgaacttgcaccgcagggttgggtgtcggtcaaggttaggcggagggcgacaggccaactccaaagacacggcgggggaggggtgcggtggagaaagcgagccgcagccaatcgcacgcgctctcccgacacctgccgccttggcgccttttctaggctactccgcgcacgcactggctgcgcgcgcagttcgcctccagcggtcttgggggagcacctcggtaggtgtacgtgcggaaggaagtgacgtagatccagagggccggccggggggtggggccgagctataagctttgggtgggaggcagcgctgccttcagaaggcgtgcggagcgcgggctgctgcattgcggactgtagaggcgcttcctagtgagtgactcccttgtcagcggcacggcccatcgtggtcctcgcgtggcgggcggaccagagcgagacgccagggcctgggtggtgcgggcggggaggcggaggggtgtcgcggagtccggggctgaggagcgcgggttgcaggtgcagcgcggtgggtgtggggagccgctgtaccctgcgcccctcgggtcctccgggccttcgcaggccagtgctaggccgcgggttcgagagtcaccacgctgaggcgcaggcttgttccgccgggagcacgtggtggcggctggaggaagtcgccccagggaacggctgtcggggtacgtgggtgaccttggggcccctcgcaggagggcgtcacagctgaaaaggacaaagctgttttctattcggttactagtgtcacggacatttagaggggcggggggagcttccaataactgcacgttggaacttcggcaccacctggtcggtttttttgccagtctctccctcttggcccagcgtgtggaatctcatttttctagggcagaataggtctgaacgctgcaggtaatactaagaacgtctctagcatctcctaagatgggagaacgtagaaatacgacctctttgtacgagctcttttagaactagctgtagagaaccagcgtgcaccctggtgttggacagctctctaaaatggtgtttgagggtaagaaaactgcatttgcaaatttttcagttagcacactttgtcccgagcgtaaaatgaaatgatctccttatacttaggcagaagactggactggattgctgttcagtttctgtgctatttttttaaaataggatttaagtgggaaatagttgtgttacagaaattctcggctattctgtgctatttttttttaaataggatttaagtgggaaatagttgtgttacagaaattctcggctacctgatacttttattctaagattagatgagttggctctgagctgtgaaatatgacctctttgacaaagacatttaagctgattcaggatgttatctacaaagaaaacgggatttagcttgtgtgggtccacttgcatttattttctgttaaggattataataaactgctttatacaggaatccaatatcagctgttttttatatagagagcataatactttttactttgagagaggatgttgtcaaggaatggtggctgtgaacctggcctgtgttgactggttagatctgtctgcctaaccccaccctaaggctaagtagttatatgcttgtggcaatgtgcttatttataatagggcaagattatgggctaaatttgggttagacaacaatgaaagttaattaaacgaccctcaggccttgggtctactatgtgtaagtgatttccttctctcccagatgagtgctatacaaaataaacttcagtgacctcaagtggttttgaccttttggttgctattcagaaaactatggaaatgaaaacctgctacctatttcctattgccttttcaatttcccaaagaaggtctcccctatgaatccatgggtagccttgaactcagatccacctgcttctgtttggagagtgataagattaaaggcaagtgccaccacacccagcaaagtaggctcttaaaactaaaacctttgcagtcgggcatggtgccacacacctttggtcccagcactggggggtaaggcagaggcaggtggatcactgagtttgaggtcagctagtgctgaagagtaagagcctgtctttaaaacatctcaacagctgggcagtcgtggtccattcctttaatcccagcacttgggaggcagaggcaagtggatttttgagttcgaggccagcctggtctacagagtgagttccaggacagccagggatacacagagaaaccctgtctcaaaaaaccaaaatataaataaataaataaagattgggagagaagtcaaggatctcataggtggtcagggagctacaactgcagtagtaaagaagtaggacttaaaagaacagggccggcactaattttgaggatctagatcgggccctcaattaaggaacttccttttgtgtgaactcagaatttgaaatgaaatgtgcttgtcagaaccattgcatggcttattttttaatgaaaagtctggctagtatctgcttatcttccagcttccagctcaaagttaaggtcatagatcaaaagaactatgtctttatcttagttgtatcttaatttttattagaattgaatggttttcctaatgtttggtaacatcaaaggtgtgtaagtaaaagtgagaaatcaagattaactttctcttggcaaagattgttgacattggtgacatcttggaccaaatgagaattgttttacttttaaatgtcccatcaacagctctcagttaggctgttctatctggtttgtcttgccatgcttgcagagtatagatttgacaatttgaaaattcaaaaagctatataaataggtatgttgctatatgtaagattttaaatgagtcagttaagacttaaagaataactgggtttattttatcttgtcaggttatcactgtgtagaccaggttgaccttgaaaacaaattctctgcttcccaagtgctgggattaaaggcgtgtgtcactagctctgacactggctactttggaactactatggtgttcacaaatgcagagttgagtgttgggattaaatggaaatttcatgtctttttttttaactttcccttctacacagggcttctctgtgtagtcctggctgtccttgtagctctagactaggctgaattcaaactcagatccacccacctaagtgctgagattaaaggcatgtgccaccactgcccagttctgaattgttggggttttttttttgttgttattcttaattttagttcgatgaattaaaatcgaaataacttgtttcttagaaaaataaggtgtaattgggttataaagccaaatttagacattaataccaacagcctgtttaggctcaaaattgttcaatcattttattagtattattattaatcatatcaacttgagacctgtttgggaaagcagaatattttagggatagctatttcagacaagcattaatgtgttagctgtttttttccccctagaatatgattaaaattggctcagggtggggccttctagttctggctctagcgattgggtctgtttctggtgaggtggtagtgataaactgtaacagaagggacaagagattgggcttctgagaacatgtatgatctggtatgtgactttaatcattaaagcatggggattcaaaaatactaatgaataggccttagaactagtcctgagtgttttgtaaaataacagtcttaattctcctagtttctggatttttttctttgtctttggatactaagtttaagcatttatttggacagagtggtgcccactagctgttctattctagtacttgggaggcaagaggcagaacgaacatggccagcttggacaacttaagaaaactgaaaggcttgccatcctagtttttcttttgattaaacacacttatattctaactagttttctctatcctttgggttttgttttgttttttatttgttttgtagctctagctggctggcttcggaattgcctgcctcccaagtgctaggattaaaggcatcacagtcactacccaattgatatcatgattcttaattcaacttctaagaacaaattatcacactctgaatctaacatggaatagcattatccatgttcagatatctttgtctcaaggctcaggtttatcctttgtagctttctttttgctatcccacctctattcagcatccagtcaaggatcactgagttggttatcagtaaattaaacattttaattaatgtctaggagacaggttatggtatagttctcagtgctgggaagttgacatggtaggatctcagttcatggccagccagaactttctggtgagatcctggttcaagcactacagagcttttctagaaaagtaactatatttaggagtaagtttgatataatgacaatcccatcgtaagccttcagtaacctgatgcattggtctctgttttaatatcaggta

SEQ ID NO: 255 - DNA, 2604 bp, Artificial Sequence
  Nucleotide sequence of the 3'-arm of targeting vector
gcattctctaacttggtaaggtactttcatctatctgaaaaaatgttcagtaaaaaacaaaacaaaaacatgacttcacccagtgagtacaagatgatacccccaattttttttttttttattatatgtatgtacactgtagctgtcttcagacacaccagaagagggcgtcagatctcatcagatggttgtgagccaccatgtggttgctgggacttgaacactggacctttggaaaagcagttgggtactcttacccactgagctatcacaccagccccaataccccaaattttgaccagccttttttttttttttttttttttttttaaatctgaactaatggtattaaggtgaaacagattgcacaaaagaggtactaggtttttctttgaggcaaggtctttctatattgcctcaggttgaccttaaactccaacttcctttttttccccaagtgctggagattgtagacagatatatacaacaccccaaaacaaatatgtttagtttcgattaagattcattatgtggggctagagggatgacttagaggttaagaacactgcctgctcttccagaggtcctgagttcaattcccagcaaccacgtggtggctcacaaccatctgtaatgggatccgatgccctctttctggtgtgtttgaagacagctacagtgtcctcatacataaaaaaaataaacaaacagatcttttaaaaaaaaaggtacagtgtacttatacattatataaatgaatgattctttaaaaaattaattatgggaaatacttatgaagaatagggtagctttggctgttttggaaacgttatataacaaggtagaactaaaatgtatgccagtaatcccagaggaatcattagccagtcagggctagtctgagcaatgtggcaagataaacccatctctttaaaaaaaaaaaaaagtattataaatagaaatgttataggaaacaggaaatagaaaccctcgaaaggctgaatgaaagagtattagtgggctggagagatggttcagcggttaagagcactatctcctgagttcagttcccagtgaccacatggtggctcacagccatctgtaatgagatctgacgccctcttctggggtgtctgaagacagcgacagtgtactcacataaaataaatacataaagactgttagttagccttcatctaccatttacagaactgggcacagaaaggagttcatcagttataaagggtaactttccatatgaatgtttgtcatattattatgcatatagtataatgaccaaactactgtaatgtcttaatatttgtatctcttttctcttttttaaaaatatcagtttggtggggaaccattgtcatacacccggtttagccttgctcggcaagtagatggagataacagtcatgtggagatgaaactggctgcagatgaagaagaaaatgccgacaataacatgaaggctagtgtcagaaaacccaagaggtttaatggaagactctgctttgcagctattgcactagtcattttcttcttgattggtaagaatgagtggccattcagaaggatttcttatgactaactagttcttagactagctagttcttagactagctagttcttgtttcttttggatgaggagatgctttgtactttaaatggcactggggctccctacctgccggcagattaggtcctgcaagatgggaaacgtttacattatggatgttttattagagatatgcaggacatttggaatagtactaagaaaggcttccagtaagacaaggtgtgcacccatgtcttaaacaggtcactgtaaaatatgacttagttgtggtaatttaaattccattaaactcaggttcataattttctattagattctcatagtttaattaaaagttttcagggataagttaaaaatgagttctgtgagtttagctctaaaacttcctgtttttaggattcatgagtggctacctgggctattgtaagcgtgtagaacaaaaagaggagtgtgtgaaactggctgaaacggaggagacagacaagtcagaaaccatggaaacagaggatgttcctacatcatctcgcttatattgggcagacctcaaaacactgttgtcagagaagttgaactccatagagtttgctgacaccatcaagtaagctcaacttcccaagttcagtcctgatggaaacgtttttgttgggggggtagggagacttgaaaggctttcagagggtcctcctgacaatgtggaactatgctgacaggaaattaggacttacctggagagcctcatagcctcctttttcttcagaatcgttttatcagttgtagtttagtgtgggatgtcagattttcttctgttctaatattccttttaaaaattttttaaaattaaaattactttttatgtattatgagtatagcctgcatatatgaatgaatgtgcattactaattacacttatctcctagtgcctacataagccttatagatggttgtgagccagcatgtgggtgctggaatccaaaatggttcttgcaagaccaaatatgttacatcccagagccattaca

SEQ ID NO: 256 - protein, 166 aa, Homo sapiens
APPRLICDSRVLERYLLEAKEAENITTGCAEHCSLNENITVPDTKVNFYAWKRMEVGQQAVEVWQGLALLSEAVLRGQALLVNSSQPWEPLQLHVDKAVSGLRSLTTLLRALGAQKEAISPPDAASAAPLRTITADTFRKLFRVYSNFLRGKLKLYTGEACRTGDR

SEQ ID NO: 257 - protein, 616 aa, Artificial Sequence
  Amino acid sequence of the fusion protein of heavy chain of anti-hTfR antibody No.3 (humanized 2) and hEPO
EVQLVQSGAEVKKPGESLKISCKGSGYSFTNYWLGWVRQMPGKGLEWMGDIYPGGDYPTYSEKFKVQVTISADKSISTAYLQWSSLKASDTAMYYCARSGNYDEVAYWGQGTLVTVSSASTKGPSVFPLAPSSKSTSGGTAALGCLVKDYFPEPVTVSWNSGALTSGVHTFPAVLQSSGLYSLSSVVTVPSSSLGTQTYICNVNHKPSNTKVDKKVEPKSCDKTHTCPPCPAPELLGGPSVFLFPPKPKDTLMISRTPEVTCVVVDVSHEDPEVKFNWYVDGVEVHNAKTKPREEQYNSTYRVVSVLTVLHQDWLNGKEYKCKVSNKALPAPIEKTISKAKGQPREPQVYTLPPSRDELTKNQVSLTCLVKGFYPSDIAVEWESNGQPENNYKTTPPVLDSDGSFFLYSKLTVDKSRWQQGNVFSCSVMHEALHNHYTQKSLSLSPGKGSAPPRLICDSRVLERYLLEAKEAENITTGCAEHCSLNENITVPDTKVNFYAWKRMEVGQQAVEVWQGLALLSEAVLRGQALLVNSSQPWEPLQLHVDKAVSGLRSLTTLLRALGAQKEAISPPDAASAAPLRTITADTFRKLFRVYSNFLRGKLKLYTGEACRTGDR

SEQ ID NO: 258 - DNA, 1931 bp, Artificial Sequence
  Nucleotide sequence encoding the amino acid sequence of fusion protein of heavy chain of anti-hTfR antibody No. 3 (humanized 2) and hEPO, synthetic sequence
acgcgtgccgccaccatgggctggagctggattctgctgttcctcctgagcgtgacagcaggagtgcacagcgaggtgcaactagtgcagtctggagcagaggtgaaaaagcccggggagtctctgaagatttcctgtaagggttctggatacagctttaccaactactggctgggatgggtgcgccagatgcccgggaaaggcctggagtggatgggggacatctaccccggcggagactaccctacatacagcgagaagttcaaggtccaggtcaccatctcagccgacaagtccatcagcaccgcctacctgcagtggagcagcctgaaggcctcggacaccgccatgtattactgtgcgagatcaggcaattacgacgaagtggcctactggggccaaggaaccctggtcaccgtctcctcagctagcaccaagggcccatcggtcttccccctggcaccctcctccaagagcacctctgggggcacagcggccctgggctgcctggtcaaggactacttccccgaaccggtgacggtgtcgtggaactcaggcgccctgaccagcggcgtgcacaccttcccggctgtcctacagtcctcaggactctactccctcagcagcgtggtgaccgtgccctccagcagcttgggcacccagacctacatctgcaacgtgaatcacaagcccagcaacaccaaggtggacaagaaagttgagcccaaatcttgtgacaaaactcacacgtgcccaccgtgcccagcacctgaactcctgggaggtccgtcagtcttcctcttccccccaaaacccaaggacaccctcatgatctcccggacccctgaggtcacatgcgtggtggtggacgtgagccacgaagaccctgaggtcaagttcaactggtacgtggacggcgtggaggtgcataatgccaagacaaagccgcgggaggagcagtacaacagcacgtaccgggtggtcagcgtcctcaccgtcctgcaccaggactggctgaatggcaaggagtacaagtgcaaggtctccaacaaagccctcccagcccccatcgagaaaaccatctccaaagccaaagggcagccccgagaaccacaggtgtacaccctgcccccatcccgggatgagctgaccaagaaccaggtcagcctgacctgcctggtcaaaggcttctatcccagcgacatcgccgtggagtgggagagcaatgggcagccggagaacaactacaagaccacgcctcccgtgctggactccgacggctccttcttcctctacagcaagctcaccgtggacaagagcaggtggcagcaggggaacgtcttctcatgctccgtgatgcatgaggctctgcacaaccactacacgcagaagagcctctccctgtctccgggtaaaggatctgccccaccacgcctcatctgtgacagccgagtcctggagaggtacctcttggaggccaaggaggccgagaatatcacgacgggctgtgctgaacactgcagcttgaatgagaatatcactgtcccagacaccaaagttaatttctatgcctggaagaggatggaggtcgggcagcaggccgtagaagtctggcagggcctggccctgctgtcggaagctgtcctgcggggccaggccctgttggtcaactcttcccagccgtgggagcccctgcagctgcatgtggataaagccgtcagtggccttcgcagcctcaccactctgcttcgggctctgggagcccagaaggaagccatctcccctccagatgcggcctcagctgctccactccgaacaatcactgctgacactttccgcaaactcttccgagtctactccaatttcctccggggaaagctgaagctgtacacaggggaggcctgcaggacaggggacagataagcggccgc

SEQ ID NO: 259 - protein, 489 aa, Homo sapiens
RPPNIVLIFADDLGYGDLGCYGHPSSTTPNLDQLAAGGLRFTDFYVPVSLCTPSRAALLTGRLPVRMGMYPGVLVPSSRGGLPLEEVTVAEVLAARGYLTGMAGKWHLGVGPEGAFLPPHQGFHRFLGIPYSHDQGPCQNLTCFPPATPCDGGCDQGLVPIPLLANLSVEAQPPWLPGLEARYMAFAHDLMADAQRQDRPFFLYYASHHTHYPQFSGQSFAERSGRGPFGDSLMELDAAVGTLMTAIGDLGLLEETLVIFTADNGPETMRMSRGGCSGLLRCGKGTTYEGGVREPALAFWPGHIAPGVTHELASSLDLLPTLAALAGAPLPNVTLDGFDLSPLLLGTGKSPRQSLFFYPSYPDEVRGVFAVRTGKYKAHFFTQGSAHSDTTADPACHASSSLTAHEPPLLYDLSKDPGENYNLLGGVAGATPEVLQALKQLQLLKAQLDAAVTFGPSQVARGEDPALQICCHPGCTPRPACCHCPDPHA

SEQ ID NO: 260 - protein, 939 aa, Artificial Sequence
  Amino acid sequence of the fusion protein of heavy chain of anti-hTfR antibody No.3 (humanized 2) and hARSA
EVQLVQSGAEVKKPGESLKISCKGSGYSFTNYWLGWVRQMPGKGLEWMGDIYPGGDYPTYSEKFKVQVTISADKSISTAYLQWSSLKASDTAMYYCARSGNYDEVAYWGQGTLVTVSSASTKGPSVFPLAPSSKSTSGGTAALGCLVKDYFPEPVTVSWNSGALTSGVHTFPAVLQSSGLYSLSSVVTVPSSSLGTQTYICNVNHKPSNTKVDKKVEPKSCDKTHTCPPCPAPELLGGPSVFLFPPKPKDTLMISRTPEVTCVVVDVSHEDPEVKFNWYVDGVEVHNAKTKPREEQYNSTYRVVSVLTVLHQDWLNGKEYKCKVSNKALPAPIEKTISKAKGQPREPQVYTLPPSRDELTKNQVSLTCLVKGFYPSDIAVEWESNGQPENNYKTTPPVLDSDGSFFLYSKLTVDKSRWQQGNVFSCSVMHEALHNHYTQKSLSLSPGKGSRPPNIVLIFADDLGYGDLGCYGHPSSTTPNLDQLAAGGLRFTDFYVPVSLCTPSRAALLTGRLPVRMGMYPGVLVPSSRGGLPLEEVTVAEVLAARGYLTGMAGKWHLGVGPEGAFLPPHQGFHRFLGIPYSHDQGPCQNLTCFPPATPCDGGCDQGLVPIPLLANLSVEAQPPWLPGLEARYMAFAHDLMADAQRQDRPFFLYYASHHTHYPQFSGQSFAERSGRGPFGDSLMELDAAVGTLMTAIGDLGLLEETLVIFTADNGPETMRMSRGGCSGLLRCGKGTTYEGGVREPALAFWPGHIAPGVTHELASSLDLLPTLAALAGAPLPNVTLDGFDLSPLLLGTGKSPRQSLFFYPSYPDEVRGVFAVRTGKYKAHFFTQGSAHSDTTADPACHASSSLTAHEPPLLYDLSKDPGENYNLLGGVAGATPEVLQALKQLQLLKAQLDAAVTFGPSQVARGEDPALQICCHPGCTPRPACCHCPDPHA

SEQ ID NO: 261 - DNA, 2900 bp, Artificial Sequence
  Nucleotide sequence encoding the amino acid sequence of fusion protein of heavy chain of anti-hTfR antibody No.3 (humanized 2) and hARSA, synthetic sequence
acgcgtgccgccaccatgggctggagctggattctgctgttcctcctgagcgtgacagcaggagtgcacagcgaggtgcaactagtgcagtctggagcagaggtgaaaaagcccggggagtctctgaagatttcctgtaagggttctggatacagctttaccaactactggctgggatgggtgcgccagatgcccgggaaaggcctggagtggatgggggacatctaccccggcggagactaccctacatacagcgagaagttcaaggtccaggtcaccatctcagccgacaagtccatcagcaccgcctacctgcagtggagcagcctgaaggcctcggacaccgccatgtattactgtgcgagatcaggcaattacgacgaagtggcctactggggccaaggaaccctggtcaccgtctcctcagctagcaccaagggcccatcggtcttccccctggcaccctcctccaagagcacctctgggggcacagcggccctgggctgcctggtcaaggactacttccccgaaccggtgacggtgtcgtggaactcaggcgccctgaccagcggcgtgcacaccttcccggctgtcctacagtcctcaggactctactccctcagcagcgtggtgaccgtgccctccagcagcttgggcacccagacctacatctgcaacgtgaatcacaagcccagcaacaccaaggtggacaagaaagttgagcccaaatcttgtgacaaaactcacacgtgcccaccgtgcccagcacctgaactcctgggaggtccgtcagtcttcctcttccccccaaaacccaaggacaccctcatgatctcccggacccctgaggtcacatgcgtggtggtggacgtgagccacgaagaccctgaggtcaagttcaactggtacgtggacggcgtggaggtgcataatgccaagacaaagccgcgggaggagcagtacaacagcacgtaccgggtggtcagcgtcctcaccgtcctgcaccaggactggctgaatggcaaggagtacaagtgcaaggtctccaacaaagccctcccagcccccatcgagaaaaccatctccaaagccaaagggcagccccgagaaccacaggtgtacaccctgcccccatcccgggatgagctgaccaagaaccaggtcagcctgacctgcctggtcaaaggcttctatcccagcgacatcgccgtggagtgggagagcaatgggcagccggagaacaactacaagaccacgcctcccgtgctggactccgacggctccttcttcctctacagcaagctcaccgtggacaagagcaggtggcagcaggggaacgtcttctcatgctccgtgatgcatgaggctctgcacaaccactacacgcagaagagcctctccctgtctccgggtaaaggatctcgtccgcccaacatcgtgctgatctttgccgacgacctcggctatggggacctgggctgctatgggcaccccagctctaccactcccaacctggaccagctggcggcgggagggctgcggttcacagacttctacgtgcctgtgtctctgtgcacaccctctagggccgccctcctgaccggccggctcccggttcggatgggcatgtaccctggcgtcctggtgcccagctcccgggggggcctgcccctggaggaggtgaccgtggccgaagtcctggctgcccgaggctacctcacaggaatggccggcaagtggcaccttggggtggggcctgagggggccttcctgcccccccatcagggcttccatcgatttctaggcatcccgtactcccacgaccagggcccctgccagaacctgacctgcttcccgccggccactccttgcgacggtggctgtgaccagggcctggtccccatcccactgttggccaacctgtccgtggaggcgcagcccccctggctgcccggactagaggcccgctacatggctttcgcccatgacctcatggccgacgcccagcgccaggatcgccccttcttcctgtactatgcctctcaccacacccactaccctcagttcagtgggcagagctttgcagagcgttcaggccgcgggccatttggggactccctgatggagctggatgcagctgtggggaccctgatgacagccataggggacctggggctgcttgaagagacgctggtcatcttcactgcagacaatggacctgagaccatgcgtatgtcccgaggcggctgctccggtctcttgcggtgtggaaagggaacgacctacgagggcggtgtccgagagcctgccttggccttctggccaggtcatatcgctcccggcgtgacccacgagctggccagctccctggacctgctgcctaccctggcagccctggctggggccccactgcccaatgtcaccttggatggctttgacctcagccccctgctgctgggcacaggcaagagccctcggcagtctctcttcttctacccgtcctacccagacgaggtccgtggggtttttgctgtgcggactggaaagtacaaggctcacttcttcacccagggctctgcccacagtgataccactgcagaccctgcctgccacgcctccagctctctgactgctcatgagcccccgctgctctatgacctgtccaaggaccctggtgagaactacaacctgctggggggtgtggccggggccaccccagaggtgctgcaagccctgaaacagcttcagctgctcaaggcccagttagacgcagctgtgaccttcggccccagccaggtggcccggggcgaggaccccgccctgcaaatctgctgtcatcctggctgcaccccccgcccagcttgctgccattgcccagatccccatgcctaagcggccgc

SEQ ID NO: 262 - protein, 279 aa, Homo sapiens
DPPAPLPLVIWHGMGDSCCNPLSMGAIKKMVEKKIPGIYVLSLEIGKTLMEDVENSFFLNVNSQVTTVCQALAKDPKLQQGYNAMGFSQGGQFLRAVAQRCPSPPMINLISVGGQHQGVFGLPRCPGESSHICDFIRKTLNAGAYSKVVQERLVQAEYWHDPIKEDVYRNHSIFLADINQERGINESYKKNLMALKKFVMVKFLNDSIVDPVDSEWFGFYRSGQAKETIPLQETSLYTQDRLGLKEMDNAGQLVFLATEGDHLQLSEEWFYAHIIPFLG

SEQ ID NO: 263 - protein, 729 aa, Artificial Sequence
  Amino acid sequence of the fusion protein of heavy chain of anti-hTfR antibody No.3 (humanized 2) and hPPT-1
EVQLVQSGAEVKKPGESLKISCKGSGYSFTNYWLGWVRQMPGKGLEWMGDIYPGGDYPTYSEKFKVQVTISADKSISTAYLQWSSLKASDTAMYYCARSGNYDEVAYWGQGTLVTVSSASTKGPSVFPLAPSSKSTSGGTAALGCLVKDYFPEPVTVSWNSGALTSGVHTFPAVLQSSGLYSLSSVVTVPSSSLGTQTYICNVNHKPSNTKVDKKVEPKSCDKTHTCPPCPAPELLGGPSVFLFPPKPKDTLMISRTPEVTCVVVDVSHEDPEVKFNWYVDGVEVHNAKTKPREEQYNSTYRVVSVLTVLHQDWLNGKEYKCKVSNKALPAPIEKTISKAKGQPREPQVYTLPPSRDELTKNQVSLTCLVKGFYPSDIAVEWESNGQPENNYKTTPPVLDSDGSFFLYSKLTVDKSRWQQGNVFSCSVMHEALHNHYTQKSLSLSPGKGSDPPAPLPLVIWHGMGDSCCNPLSMGAIKKMVEKKIPGIYVLSLEIGKTLMEDVENSFFLNVNSQVTTVCQALAKDPKLQQGYNAMGFSQGGQFLRAVAQRCPSPPMINLISVGGQHQGVFGLPRCPGESSHICDFIRKTLNAGAYSKVVQERLVQAEYWHDPIKEDVYRNHSIFLADINQERGINESYKKNLMALKKFVMVKFLNDSIVDPVDSEWFGFYRSGQAKETIPLQETSLYTQDRLGLKEMDNAGQLVFLATEGDHLQLSEEWFYAHIIPFLG

SEQ ID NO: 264 - DNA, 2270 bp, Artificial Sequence
  Nucleotide sequence encoding the amino acid sequence of fusion protein of heavy chain of anti-hTfR antibody No.3 (humanized 2) and hPPT-1, synthetic sequence
acgcgtgccgccaccatgggctggagctggattctgctgttcctcctgagcgtgacagcaggagtgcacagcgaggtgcaactagtgcagtctggagcagaggtgaaaaagcccggggagtctctgaagatttcctgtaagggttctggatacagctttaccaactactggctgggatgggtgcgccagatgcccgggaaaggcctggagtggatgggggacatctaccccggcggagactaccctacatacagcgagaagttcaaggtccaggtcaccatctcagccgacaagtccatcagcaccgcctacctgcagtggagcagcctgaaggcctcggacaccgccatgtattactgtgcgagatcaggcaattacgacgaagtggcctactggggccaaggaaccctggtcaccgtctcctcagctagcaccaagggcccatcggtcttccccctggcaccctcctccaagagcacctctgggggcacagcggccctgggctgcctggtcaaggactacttccccgaaccggtgacggtgtcgtggaactcaggcgccctgaccagcggcgtgcacaccttcccggctgtcctacagtcctcaggactctactccctcagcagcgtggtgaccgtgccctccagcagcttgggcacccagacctacatctgcaacgtgaatcacaagcccagcaacaccaaggtggacaagaaagttgagcccaaatcttgtgacaaaactcacacgtgcccaccgtgcccagcacctgaactcctgggaggtccgtcagtcttcctcttccccccaaaacccaaggacaccctcatgatctcccggacccctgaggtcacatgcgtggtggtggacgtgagccacgaagaccctgaggtcaagttcaactggtacgtggacggcgtggaggtgcataatgccaagacaaagccgcgggaggagcagtacaacagcacgtaccgggtggtcagcgtcctcaccgtcctgcaccaggactggctgaatggcaaggagtacaagtgcaaggtctccaacaaagccctcccagcccccatcgagaaaaccatctccaaagccaaagggcagccccgagaaccacaggtgtacaccctgcccccatcccgggatgagctgaccaagaaccaggtcagcctgacctgcctggtcaaaggcttctatcccagcgacatcgccgtggagtgggagagcaatgggcagccggagaacaactacaagaccacgcctcccgtgctggactccgacggctccttcttcctctacagcaagctcaccgtggacaagagcaggtggcagcaggggaacgtcttctcatgctccgtgatgcatgaggctctgcacaaccactacacgcagaagagcctctccctgtctccgggtaaaggatctgacccgccggcgccgctgccgttggtgatctggcatgggatgggagacagctgttgcaatcccttaagcatgggtgctattaaaaaaatggtggagaagaaaatacctggaatttacgtcttatctttagagattgggaagaccctgatggaggacgtggagaacagcttcttcttgaatgtcaattcccaagtaacaacagtgtgtcaggcacttgctaaagatcctaaattgcagcaaggctacaatgctatgggattctcccagggaggccaatttctgagggcagtggctcagagatgcccttcacctcccatgatcaatctgatctcggttgggggacaacatcaaggtgtttttggactccctcgatgcccaggagagagctctcacatctgtgacttcatccgaaaaacactgaatgctggggcgtactccaaagttgttcaggaacgcctcgtgcaagccgaatactggcatgaccccataaaggaggatgtgtatcgcaaccacagcatcttcttggcagatataaatcaggagcggggtatcaatgagtcctacaagaaaaacctgatggccctgaagaagtttgtgatggtgaaattcctcaatgattccattgtggaccctgtagattcggagtggtttggattttacagaagtggccaagccaaggaaaccattcccttacaggagacctccctgtacacacaggaccgcctggggctaaaggaaatggacaatgcaggacagctagtgtttctggctacagaaggggaccatcttcagttgtctgaagaatggttttatgcccacatcataccattccttggataagcggccgc

SEQ ID NO: 265 - protein, 544 aa, Homo sapiens
SYSPEPDQRRTLPPGWVSLGRADPEEELSLTFALRQQNVERLSELVQAVSDPSSPQYGKYLTLENVADLVRPSPLTLHTVQKWLLAAGAQKCHSVITQDFLTCWLSIRQAELLLPGAEFHHYVGGPTETHVVRSPHPYQLPQALAPHVDFVGGLHHFPPTSSLRQRPEPQVTGTVGLHLGVTPSVIRKRYNLTSQDVGSGTSNNSQACAQFLEQYFHDSDLAQFMRLFGGNFAHQASVARVVGQQGRGRAGIEASLDVQYLMSAGANISTWVYSSPGRHEGQEPFLQWLMLLSNESALPHVHTVSYGDDEDSLSSAYIQRVNTELMKAAARGLTLLFASGDSGAGCWSVSGRHQFRPTFPASSPYVTTVGGTSFQEPFLITNEIVDYISGGGFSNVFPRPSYQEEAVTKFLSSSPHLPPSSYFNASGRAYPDVAALSDGYWVVSNRVPIPWVSGTSASTPVFGGILSLINEHRILSGRPPLGFLNPRLYQQHGAGLFDVTRGCHESCLDEEVEGQGFCSGPGWDPVTGWGTPNFPALLKTLLNP

SEQ ID NO: 266 - protein, 994 aa, Artificial Sequence
  Amino acid sequence of the fusion protein of heavy chain of anti-hTfR antibody No.3 (humanized 2) and hTPP-1
EVQLVQSGAEVKKPGESLKISCKGSGYSFTNYWLGWVRQMPGKGLEWMGDIYPGGDYPTYSEKFKVQVTISADKSISTAYLQWSSLKASDTAMYYCARSGNYDEVAYWGQGTLVTVSSASTKGPSVFPLAPSSKSTSGGTAALGCLVKDYFPEPVTVSWNSGALTSGVHTFPAVLQSSGLYSLSSVVTVPSSSLGTQTYICNVNHKPSNTKVDKKVEPKSCDKTHTCPPCPAPELLGGPSVFLFPPKPKDTLMISRTPEVTCVVVDVSHEDPEVKFNWYVDGVEVHNAKTKPREEQYNSTYRVVSVLTVLHQDWLNGKEYKCKVSNKALPAPIEKTISKAKGQPREPQVYTLPPSRDELTKNQVSLTCLVKGFYPSDIAVEWESNGQPENNYKTTPPVLDSDGSFFLYSKLTVDKSRWQQGNVFSCSVMHEALHNHYTQKSLSLSPGKGSSYSPEPDQRRTLPPGWVSLGRADPEEELSLTFALRQQNVERLSELVQAVSDPSSPQYGKYLTLENVADLVRPSPLTLHTVQKWLLAAGAQKCHSVITQDFLTCWLSIRQAELLLPGAEFHHYVGGPTETHVVRSPHPYQLPQALAPHVDFVGGLHHFPPTSSLRQRPEPQVTGTVGLHLGVTPSVIRKRYNLTSQDVGSGTSNNSQACAQFLEQYFHDSDLAQFMRLFGGNFAHQASVARVVGQQGRGRAGIEASLDVQYLMSAGANISTWVYSSPGRHEGQEPFLQWLMLLSNESALPHVHTVSYGDDEDSLSSAYIQRVNTELMKAAARGLTLLFASGDSGAGCWSVSGRHQFRPTFPASSPYVTTVGGTSFQEPFLITNEIVDYISGGGFSNVFPRPSYQEEAVTKFLSSSPHLPPSSYFNASGRAYPDVAALSDGYWVVSNRVPIPWVSGTSASTPVFGGILSLINEHRILSGRPPLGFLNPRLYQQHGAGLFDVTRGCHESCLDEEVEGQGFCSGPGWDPVTGWGTPNFPALLKTLLNP

SEQ ID NO: 267 - DNA, 3065 bp, Artificial Sequence
  Nucleotide sequence encoding the amino acid sequence of fusion protein of heavy chain of anti-hTfR antibody No.3 (humanized 2) and hTPP-1, synthetic sequence
acgcgtgccgccaccatgggctggagctggattctgctgttcctcctgagcgtgacagcaggagtgcacagcgaggtgcaactagtgcagtctggagcagaggtgaaaaagcccggggagtctctgaagatttcctgtaagggttctggatacagctttaccaactactggctgggatgggtgcgccagatgcccgggaaaggcctggagtggatgggggacatctaccccggcggagactaccctacatacagcgagaagttcaaggtccaggtcaccatctcagccgacaagtccatcagcaccgcctacctgcagtggagcagcctgaaggcctcggacaccgccatgtattactgtgcgagatcaggcaattacgacgaagtggcctactggggccaaggaaccctggtcaccgtctcctcagctagcaccaagggcccatcggtcttccccctggcaccctcctccaagagcacctctgggggcacagcggccctgggctgcctggtcaaggactacttccccgaaccggtgacggtgtcgtggaactcaggcgccctgaccagcggcgtgcacaccttcccggctgtcctacagtcctcaggactctactccctcagcagcgtggtgaccgtgccctccagcagcttgggcacccagacctacatctgcaacgtgaatcacaagcccagcaacaccaaggtggacaagaaagttgagcccaaatcttgtgacaaaactcacacgtgcccaccgtgcccagcacctgaactcctgggaggtccgtcagtcttcctcttccccccaaaacccaaggacaccctcatgatctcccggacccctgaggtcacatgcgtggtggtggacgtgagccacgaagaccctgaggtcaagttcaactggtacgtggacggcgtggaggtgcataatgccaagacaaagccgcgggaggagcagtacaacagcacgtaccgggtggtcagcgtcctcaccgtcctgcaccaggactggctgaatggcaaggagtacaagtgcaaggtctccaacaaagccctcccagcccccatcgagaaaaccatctccaaagccaaagggcagccccgagaaccacaggtgtacaccctgcccccatcccgggatgagctgaccaagaaccaggtcagcctgacctgcctggtcaaaggcttctatcccagcgacatcgccgtggagtgggagagcaatgggcagccggagaacaactacaagaccacgcctcccgtgctggactccgacggctccttcttcctctacagcaagctcaccgtggacaagagcaggtggcagcaggggaacgtcttctcatgctccgtgatgcatgaggctctgcacaaccactacacgcagaagagcctctccctgtctccgggtaaaggatctagttacagcccggagcccgaccagcggaggacgctgcccccaggctgggtgtccctgggccgtgcggaccctgaggaagagctgagtctcacctttgccctgagacagcagaatgtggaaagactctcggagctggtgcaggctgtgtcagatcccagctctcctcaatacggaaaatacctgaccctagagaatgtggctgatctggtgaggccatccccactgaccctccacacggtgcaaaaatggctcttggcagccggagcccagaagtgccattctgtgatcacacaggactttctgacttgctggctgagcatccgacaagcagagctgctgctccctggggctgagtttcatcactatgtgggaggacctacggaaacccatgttgtaaggtccccacatccctaccagcttccacaggccttggccccccatgtggactttgtggggggactgcaccattttcccccaacatcatccctgaggcaacgtcctgagccgcaggtgacagggactgtaggcctgcatctgggggtaaccccctctgtgatccgtaagcgatacaacttgacctcacaagacgtgggctctggcaccagcaataacagccaagcctgtgcccagttcctggagcagtatttccatgactcagacctggctcagttcatgcgcctcttcggtggcaactttgcacatcaggcatcagtagcccgtgtggttggacaacagggccggggccgggccgggattgaggccagtctagatgtgcagtacctgatgagtgctggtgccaacatctccacctgggtctacagtagccctggccggcatgagggacaggagcccttcctgcagtggctcatgctgctcagtaatgagtcagccctgccacatgtgcatactgtgagctatggagatgatgaggactccctcagcagcgcctacatccagcgggtcaacactgagctcatgaaggctgctgctcggggtctcaccctgctcttcgcctcaggtgacagtggggccgggtgttggtctgtctctggaagacaccagttccgccctaccttccctgcctccagcccctatgtcaccacagtgggaggcacatccttccaggaacctttcctcatcacaaatgaaattgttgactatatcagtggtggtggcttcagcaatgtgttcccacggccttcataccaggaggaagctgtaacgaagttcctgagctctagcccccacctgccaccatccagttacttcaatgccagtggccgtgcctacccagatgtggctgcactttctgatggctactgggtggtcagcaacagagtgcccattccatgggtgtccggaacctcggcctctactccagtgtttgggggtatcctatccttgatcaatgagcacagaatccttagtggccgcccccctcttggctttctcaacccaaggctctaccagcagcatggggcaggactctttgatgtaacccgtggctgccatgagtcctgtctggatgaagaggtagagggccagggtttctgctctggtcctggctgggaccctgtaacaggctggggaacacccaacttcccagctttgctgaagactctactcaacccctaagcggccgc

SEQ ID NO: 268 - protein, 628 aa, Homo sapiens
AEAPHLVHVDAARALWPLRRFWRSTGFCPPLPHSQADQYVLSWDQQLNLAYVGAVPHRGIKQVRTHWLLELVTTRGSTGRGLSYNFTHLDGYLDLLRENQLLPGFELMGSASGHFTDFEDKQQVFEWKDLVSSLARRYIGRYGLAHVSKWNFETWNEPDHHDFDNVSMTMQGFLNYYDACSEGLRAASPALRLGGPGDSFHTPPRSPLSWGLLRHCHDGTNFFTGEAGVRLDYISLHRKGARSSISILEQEKVVAQQIRQLFPKFADTPIYNDEADPLVGWSLPQPWRADVTYAAMVVKVIAQHQNLLLANTTSAFPYALLSNDNAFLSYHPHPFAQRTLTARFQVNNTRPPHVQLLRKPVLTAMGLLALLDEEQLWAEVSQAGTVLDSNHTVGVLASAHRPQGPADAWRAAVLIYASDDTRAHPNRSVAVTLRLRGVPPGPGLVYVTRYLDNGLCSPDGEWRRLGRPVFPTAEQFRRMRAAEDPVAAAPRPLPAGGRLTLRPALRLPSLLLVHVCARPEKPPGQVTRLRALPLTQGQLVLVWSDEHVGSKCLWTYEIQFSQDGKAYTPVSRKPSTFNLFVFSPDTGAVSGSYRVRALDYWARPGPFSDPVPYLEVPVPRGPPSPGNP

SEQ ID NO: 269 - protein, 1078 aa, Artificial Sequence
  Amino acid sequence of the fusion protein of heavy chain of anti-hTfR antibody No.3 (humanized 2) and hIDUA
EVQLVQSGAEVKKPGESLKISCKGSGYSFTNYWLGWVRQMPGKGLEWMGDIYPGGDYPTYSEKFKVQVTISADKSISTAYLQWSSLKASDTAMYYCARSGNYDEVAYWGQGTLVTVSSASTKGPSVFPLAPSSKSTSGGTAALGCLVKDYFPEPVTVSWNSGALTSGVHTFPAVLQSSGLYSLSSVVTVPSSSLGTQTYICNVNHKPSNTKVDKKVEPKSCDKTHTCPPCPAPELLGGPSVFLFPPKPKDTLMISRTPEVTCVVVDVSHEDPEVKFNWYVDGVEVHNAKTKPREEQYNSTYRVVSVLTVLHQDWLNGKEYKCKVSNKALPAPIEKTISKAKGQPREPQVYTLPPSRDELTKNQVSLTCLVKGFYPSDIAVEWESNGQPENNYKTTPPVLDSDGSFFLYSKLTVDKSRWQQGNVFSCSVMHEALHNHYTQKSLSLSPGKGSAEAPHLVHVDAARALWPLRRFWRSTGFCPPLPHSQADQYVLSWDQQLNLAYVGAVPHRGIKQVRTHWLLELVTTRGSTGRGLSYNFTHLDGYLDLLRENQLLPGFELMGSASGHFTDFEDKQQVFEWKDLVSSLARRYIGRYGLAHVSKWNFETWNEPDHHDFDNVSMTMQGFLNYYDACSEGLRAASPALRLGGPGDSFHTPPRSPLSWGLLRHCHDGTNFFTGEAGVRLDYISLHRKGARSSISILEQEKVVAQQIRQLFPKFADTPIYNDEADPLVGWSLPQPWRADVTYAAMVVKVIAQHQNLLLANTTSAFPYALLSNDNAFLSYHPHPFAQRTLTARFQVNNTRPPHVQLLRKPVLTAMGLLALLDEEQLWAEVSQAGTVLDSNHTVGVLASAHRPQGPADAWRAAVLIYASDDTRAHPNRSVAVTLRLRGVPPGPGLVYVTRYLDNGLCSPDGEWRRLGRPVFPTAEQFRRMRAAEDPVAAAPRPLPAGGRLTLRPALRLPSLLLVHVCARPEKPPGQVTRLRALPLTQGQLVLVWSDEHVGSKCLWTYEIQFSQDGKAYTPVSRKPSTFNLFVFSPDTGAVSGSYRVRALDYWARPGPFSDPVPYLEVPVPRGPPSPGNP

SEQ ID NO: 270 - DNA, 3317 bp, Artificial Sequence
  Nucleotide sequence encoding the amino acid sequence of fusion protein of heavy chain of anti-hTfR antibody No.3 (humanized 2) and hIDUA, synthetic sequence
acgcgtgccgccaccatgggctggagctggattctgctgttcctcctgagcgtgacagcaggagtgcacagcgaggtgcaactagtgcagtctggagcagaggtgaaaaagcccggggagtctctgaagatttcctgtaagggttctggatacagctttaccaactactggctgggatgggtgcgccagatgcccgggaaaggcctggagtggatgggggacatctaccccggcggagactaccctacatacagcgagaagttcaaggtccaggtcaccatctcagccgacaagtccatcagcaccgcctacctgcagtggagcagcctgaaggcctcggacaccgccatgtattactgtgcgagatcaggcaattacgacgaagtggcctactggggccaaggaaccctggtcaccgtctcctcagctagcaccaagggcccatcggtcttccccctggcaccctcctccaagagcacctctgggggcacagcggccctgggctgcctggtcaaggactacttccccgaaccggtgacggtgtcgtggaactcaggcgccctgaccagcggcgtgcacaccttcccggctgtcctacagtcctcaggactctactccctcagcagcgtggtgaccgtgccctccagcagcttgggcacccagacctacatctgcaacgtgaatcacaagcccagcaacaccaaggtggacaagaaagttgagcccaaatcttgtgacaaaactcacacgtgcccaccgtgcccagcacctgaactcctgggaggtccgtcagtcttcctcttccccccaaaacccaaggacaccctcatgatctcccggacccctgaggtcacatgcgtggtggtggacgtgagccacgaagaccctgaggtcaagttcaactggtacgtggacggcgtggaggtgcataatgccaagacaaagccgcgggaggagcagtacaacagcacgtaccgggtggtcagcgtcctcaccgtcctgcaccaggactggctgaatggcaaggagtacaagtgcaaggtctccaacaaagccctcccagcccccatcgagaaaaccatctccaaagccaaagggcagccccgagaaccacaggtgtacaccctgcccccatcccgggatgagctgaccaagaaccaggtcagcctgacctgcctggtcaaaggcttctatcccagcgacatcgccgtggagtgggagagcaatgggcagccggagaacaactacaagaccacgcctcccgtgctggactccgacggctccttcttcctctacagcaagctcaccgtggacaagagcaggtggcagcaggggaacgtcttctcatgctccgtgatgcatgaggctctgcacaaccactacacgcagaagagcctctccctgtctccgggtaaaggatctgccgaggccccgcacctggtgcacgtggacgcggcccgcgcgctgtggcccctgcggcgcttctggaggagcacaggcttctgccccccgctgccacacagccaggctgaccagtacgtcctcagctgggaccagcagctcaacctcgcctatgtgggcgccgtccctcaccgcggcatcaagcaggtccggacccactggctgctggagcttgtcaccaccagggggtccactggacggggcctgagctacaacttcacccacctggacgggtacttggaccttctcagggagaaccagctcctcccagggtttgagctgatgggcagcgcctcgggccacttcactgactttgaggacaagcagcaggtgtttgagtggaaggacttggtctccagcctggccaggagatacatcggtaggtacggactggcgcatgtttccaagtggaacttcgagacgtggaatgagccagaccaccacgactttgacaacgtctccatgaccatgcaaggcttcctgaactactacgatgcctgctcggagggtctgcgcgccgccagccccgccctgcggctgggaggccccggcgactccttccacaccccaccgcgatccccgctgagctggggcctcctgcgccactgccacgacggtaccaacttcttcactggggaggcgggcgtgcggctggactacatctccctccacaggaagggtgcgcgcagctccatctccatcctggagcaggagaaggtcgtcgcgcagcagatccggcagctcttccccaagttcgcggacacccccatttacaacgacgaggcggacccgctggtgggctggtccctgccacagccgtggagggcggacgtgacctacgcggccatggtggtgaaggtcatcgcgcagcatcagaacctgctactggccaacaccacctccgccttcccctacgcgctcctgagcaacgacaatgccttcctgagctaccacccgcaccccttcgcgcagcgcacgctcaccgcgcgcttccaggtcaacaacacccgcccgccgcacgtgcagctgttgcgcaagccggtgctcacggccatggggctgctggcgctgctggatgaggagcagctctgggccgaagtgtcgcaggccgggaccgtcctggacagcaaccacacggtgggcgtcctggccagcgcccaccgcccccagggcccggccgacgcctggcgcgccgcggtgctgatctacgcgagcgacgacacccgcgcccaccccaaccgcagcgtcgcggtgaccctgcggctgcgcggggtgccccccggcccgggcctggtctacgtcacgcgctacctggacaacgggctctgcagccccgacggcgagtggcggcgcctgggccggcccgtcttccccacggcagagcagttccggcgcatgcgcgcggctgaggacccggtggccgcggcgccccgccccttacccgccggtggccgcctgaccctgcgccccgcgctgcggctgccgtcgcttttgctggtgcacgtgtgtgcgcgccccgagaagccgcccgggcaggtcacgcggctccgcgccctgcccctgacccaagggcagctggttctggtctggtcggatgaacacgtgggctccaagtgcctgtggacatacgagatccagttctctcaggacggtaaggcgtacaccccggtcagcaggaagccatcgaccttcaacctctttgtgttcagcccagacacaggtgctgtctctggctcctaccgagttcgagccctggactactgggcccgaccaggccccttctcggaccctgtgccgtacctggaggtccctgtgccaagagggcccccatccccgggcaatccataagcggccgc

SEQ ID NO: 271 - protein, 235 aa, Homo sapiens
LPAQVAFTPYAPEPGSTCRLREYYDQTAQMCCSKCSPGQHAKVFCTKTSDTVCDSCEDSTYTQLWNWVPECLSCGSRCSSDQVETQACTREQNRICTCRPGWYCALSKQEGCRLCAPLRKCRPGFGVARPGTETSDVVCKPCAPGTFSNTTSSTDICRPHQICNVVAIPGNASMDAVCTSTSPTRSMAPGAVHLPQPVSTRSQHTQPTPEPSTAPSTSFLLPMGPSPPAEGSTGD

SEQ ID NO: 272 - protein, 685 aa, Artificial Sequence
  Amino acid sequence of the fusion protein of heavy chain of anti-hTfR antibody No.3 (humanized 2) and hTNF-alpha receptor
EVQLVQSGAEVKKPGESLKISCKGSGYSFTNYWLGWVRQMPGKGLEWMGDIYPGGDYPTYSEKFKVQVTISADKSISTAYLQWSSLKASDTAMYYCARSGNYDEVAYWGQGTLVTVSSASTKGPSVFPLAPSSKSTSGGTAALGCLVKDYFPEPVTVSWNSGALTSGVHTFPAVLQSSGLYSLSSVVTVPSSSLGTQTYICNVNHKPSNTKVDKKVEPKSCDKTHTCPPCPAPELLGGPSVFLFPPKPKDTLMISRTPEVTCVVVDVSHEDPEVKFNWYVDGVEVHNAKTKPREEQYNSTYRVVSVLTVLHQDWLNGKEYKCKVSNKALPAPIEKTISKAKGQPREPQVYTLPPSRDELTKNQVSLTCLVKGFYPSDIAVEWESNGQPENNYKTTPPVLDSDGSFFLYSKLTVDKSRWQQGNVFSCSVMHEALHNHYTQKSLSLSPGKGSLPAQVAFTPYAPEPGSTCRLREYYDQTAQMCCSKCSPGQHAKVFCTKTSDTVCDSCEDSTYTQLWNWVPECLSCGSRCSSDQVETQACTREQNRICTCRPGWYCALSKQEGCRLCAPLRKCRPGFGVARPGTETSDVVCKPCAPGTFSNTTSSTDICRPHQICNVVAIPGNASMDAVCTSTSPTRSMAPGAVHLPQPVSTRSQHTQPTPEPSTAPSTSFLLPMGPSPPAEGSTGD

SEQ ID NO: 273 - DNA, 2138 bp, Artificial Sequence
  Nucleotide sequence encoding the amino acid sequence of fusion protein of heavy chain of anti-hTfR antibody No.3 (humanized 2) and hTNF-alpha receptor, synthetic sequence
acgcgtgccgccaccatgggctggagctggattctgctgttcctcctgagcgtgacagcaggagtgcacagcgaggtgcaactagtgcagtctggagcagaggtgaaaaagcccggggagtctctgaagatttcctgtaagggttctggatacagctttaccaactactggctgggatgggtgcgccagatgcccgggaaaggcctggagtggatgggggacatctaccccggcggagactaccctacatacagcgagaagttcaaggtccaggtcaccatctcagccgacaagtccatcagcaccgcctacctgcagtggagcagcctgaaggcctcggacaccgccatgtattactgtgcgagatcaggcaattacgacgaagtggcctactggggccaaggaaccctggtcaccgtctcctcagctagcaccaagggcccatcggtcttccccctggcaccctcctccaagagcacctctgggggcacagcggccctgggctgcctggtcaaggactacttccccgaaccggtgacggtgtcgtggaactcaggcgccctgaccagcggcgtgcacaccttcccggctgtcctacagtcctcaggactctactccctcagcagcgtggtgaccgtgccctccagcagcttgggcacccagacctacatctgcaacgtgaatcacaagcccagcaacaccaaggtggacaagaaagttgagcccaaatcttgtgacaaaactcacacgtgcccaccgtgcccagcacctgaactcctgggaggtccgtcagtcttcctcttccccccaaaacccaaggacaccctcatgatctcccggacccctgaggtcacatgcgtggtggtggacgtgagccacgaagaccctgaggtcaagttcaactggtacgtggacggcgtggaggtgcataatgccaagacaaagccgcgggaggagcagtacaacagcacgtaccgggtggtcagcgtcctcaccgtcctgcaccaggactggctgaatggcaaggagtacaagtgcaaggtctccaacaaagccctcccagcccccatcgagaaaaccatctccaaagccaaagggcagccccgagaaccacaggtgtacaccctgcccccatcccgggatgagctgaccaagaaccaggtcagcctgacctgcctggtcaaaggcttctatcccagcgacatcgccgtggagtgggagagcaatgggcagccggagaacaactacaagaccacgcctcccgtgctggactccgacggctccttcttcctctacagcaagctcaccgtggacaagagcaggtggcagcaggggaacgtcttctcatgctccgtgatgcatgaggctctgcacaaccactacacgcagaagagcctctccctgtctccgggtaaaggatctttgcccgcccaggtggcatttacaccctacgccccggagcccgggagcacatgccggctcagagaatactatgaccagacagctcagatgtgctgcagcaagtgctcgccgggccaacatgcaaaagtcttctgtaccaagacctcggacaccgtgtgtgactcctgtgaggacagcacatacacccagctctggaactgggttcccgagtgcttgagctgtggctcccgctgtagctctgaccaggtggaaactcaagcctgcactcgggaacagaaccgcatctgcacctgcaggcccggctggtactgcgcgctgagcaagcaggaggggtgccggctgtgcgcgccgctgcgcaagtgccgcccgggcttcggcgtggccagaccaggaactgaaacatcagacgtggtgtgcaagccctgtgccccggggacgttctccaacacgacttcatccacggatatttgcaggccccaccaaatctgtaacgtggtggccatccctgggaatgcaagcatggatgcagtctgcacgtccacgtcccccacccggagtatggccccaggggcagtacacttaccccagccagtgtccacacgatcccaacacacgcagccaactccagaacccagcactgctccaagcacctccttcctgctcccaatgggccccagccccccagctgaagggagcactggcgactaagcggccgc

SEQ ID NO: 274 - protein, 482 aa, Homo sapiens
RPRNALLLLADDGGFESGAYNNSAIATPHLDALARRSLLFRNAFTSVSSCSPSRASLLTGLPQHQNGMYGLHQDVHHFNSFDKVRSLPLLLSQAGVRTGIIGKKHVGPETVYPFDFAYTEENGSVLQVGRNITRIKLLVRKFLQTQDDRPFFLYVAFHDPHRCGHSQPQYGTFCEKFGNGESGMGRIPDWTPQAYDPLDVLVPYFVPNTPAARADLAAQYTTVGRMDQGVGLVLQELRDAGVLNDTLVIFTSDNGIPFPSGRTNLYWPGTAEPLLVSSPEHPKRWGQVSEAYVSLLDLTPTILDWFSIPYPSYAIFGSKTIHLTGRSLLPALEAEPLWATVFGSQSHHEVTMSYPMRSVQHRHFRLVHNLNFKMPFPIDQDFYVSPTFQDLLNRTTAGQPTGWYKDLRHYYYRARWELYDRSRDPHETQNLATDPRFAQLLEMLRDQLAKWQWETHDPWVCAPDGVLEEKLSPQCQPLHNEL

SEQ ID NO: 275 - protein, 932 aa, Artificial Sequence
  Amino acid sequence of the fusion protein of heavy chain of anti-hTfR antibody No.3 (humanized 2) and hSGSH
EVQLVQSGAEVKKPGESLKISCKGSGYSFTNYWLGWVRQMPGKGLEWMGDIYPGGDYPTYSEKFKVQVTISADKSISTAYLQWSSLKASDTAMYYCARSGNYDEVAYWGQGTLVTVSSASTKGPSVFPLAPSSKSTSGGTAALGCLVKDYFPEPVTVSWNSGALTSGVHTFPAVLQSSGLYSLSSVVTVPSSSLGTQTYICNVNHKPSNTKVDKKVEPKSCDKTHTCPPCPAPELLGGPSVFLFPPKPKDTLMISRTPEVTCVVVDVSHEDPEVKFNWYVDGVEVHNAKTKPREEQYNSTYRVVSVLTVLHQDWLNGKEYKCKVSNKALPAPIEKTISKAKGQPREPQVYTLPPSRDELTKNQVSLTCLVKGFYPSDIAVEWESNGQPENNYKTTPPVLDSDGSFFLYSKLTVDKSRWQQGNVFSCSVMHEALHNHYTQKSLSLSPGKGSRPRNALLLLADDGGFESGAYNNSAIATPHLDALARRSLLFRNAFTSVSSCSPSRASLLTGLPQHQNGMYGLHQDVHHFNSFDKVRSLPLLLSQAGVRTGIIGKKHVGPETVYPFDFAYTEENGSVLQVGRNITRIKLLVRKFLQTQDDRPFFLYVAFHDPHRCGHSQPQYGTFCEKFGNGESGMGRIPDWTPQAYDPLDVLVPYFVPNTPAARADLAAQYTTVGRMDQGVGLVLQELRDAGVLNDTLVIFTSDNGIPFPSGRTNLYWPGTAEPLLVSSPEHPKRWGQVSEAYVSLLDLTPTILDWFSIPYPSYAIFGSKTIHLTGRSLLPALEAEPLWATVFGSQSHHEVTMSYPMRSVQHRHFRLVHNLNFKMPFPIDQDFYVSPTFQDLLNRTTAGQPTGWYKDLRHYYYRARWELYDRSRDPHETQNLATDPRFAQLLEMLRDQLAKWQWETHDPWVCAPDGVLEEKLSPQCQPLHNEL

SEQ ID NO: 276 - DNA, 2879 bp, Artificial Sequence
  Nucleotide sequence encoding the amino acid sequence of fusion protein of heavy chain of anti-hTfR antibody No.3 (humanized 2) and hSGSH, synthetic sequence
acgcgtgccgccaccatgggctggagctggattctgctgttcctcctgagcgtgacagcaggagtgcacagcgaggtgcaactagtgcagtctggagcagaggtgaaaaagcccggggagtctctgaagatttcctgtaagggttctggatacagctttaccaactactggctgggatgggtgcgccagatgcccgggaaaggcctggagtggatgggggacatctaccccggcggagactaccctacatacagcgagaagttcaaggtccaggtcaccatctcagccgacaagtccatcagcaccgcctacctgcagtggagcagcctgaaggcctcggacaccgccatgtattactgtgcgagatcaggcaattacgacgaagtggcctactggggccaaggaaccctggtcaccgtctcctcagctagcaccaagggcccatcggtcttccccctggcaccctcctccaagagcacctctgggggcacagcggccctgggctgcctggtcaaggactacttccccgaaccggtgacggtgtcgtggaactcaggcgccctgaccagcggcgtgcacaccttcccggctgtcctacagtcctcaggactctactccctcagcagcgtggtgaccgtgccctccagcagcttgggcacccagacctacatctgcaacgtgaatcacaagcccagcaacaccaaggtggacaagaaagttgagcccaaatcttgtgacaaaactcacacgtgcccaccgtgcccagcacctgaactcctgggaggtccgtcagtcttcctcttccccccaaaacccaaggacaccctcatgatctcccggacccctgaggtcacatgcgtggtggtggacgtgagccacgaagaccctgaggtcaagttcaactggtacgtggacggcgtggaggtgcataatgccaagacaaagccgcgggaggagcagtacaacagcacgtaccgggtggtcagcgtcctcaccgtcctgcaccaggactggctgaatggcaaggagtacaagtgcaaggtctccaacaaagccctcccagcccccatcgagaaaaccatctccaaagccaaagggcagccccgagaaccacaggtgtacaccctgcccccatcccgggatgagctgaccaagaaccaggtcagcctgacctgcctggtcaaaggcttctatcccagcgacatcgccgtggagtgggagagcaatgggcagccggagaacaactacaagaccacgcctcccgtgctggactccgacggctccttcttcctctacagcaagctcaccgtggacaagagcaggtggcagcaggggaacgtcttctcatgctccgtgatgcatgaggctctgcacaaccactacacgcagaagagcctctccctgtctccgggtaaaggatctcgtccccggaacgcactgctgctcctcgcggatgacggaggctttgagagtggcgcgtacaacaacagcgccatcgccaccccgcacctggacgccttggcccgccgcagcctcctctttcgcaatgccttcacctcggtcagcagctgctctcccagccgcgccagcctcctcactggcctgccccagcatcagaatgggatgtacgggctgcaccaggacgtgcaccacttcaactccttcgacaaggtgcggagcctgccgctgctgctcagccaagctggtgtgcgcacaggcatcatcgggaagaagcacgtggggccggagaccgtgtacccgtttgactttgcgtacacggaggagaatggctccgtcctccaggtggggcggaacatcactagaattaagctgctcgtccggaaattcctgcagactcaggatgaccggcctttcttcctctacgtcgccttccacgacccccaccgctgtgggcactcccagccccagtacggaaccttctgtgagaagtttggcaacggagagagcggcatgggtcgtatcccagactggaccccccaggcctacgacccactggacgtgctggtgccttacttcgtccccaacaccccggcagcccgagccgacctggccgctcagtacaccaccgtcggccgcatggaccaaggagttggactggtgctccaggagctgcgtgacgccggtgtcctgaacgacacactggtgatcttcacgtccgacaacggtatccccttccccagcggcaggaccaacctgtactggccgggcactgctgaacccttactggtgtcatccccggagcacccaaaacgctggggccaagtcagcgaggcctacgtgagcctcctagacctcacgcccaccatcttggattggttctcgatcccgtaccccagctacgccatctttggctcgaagaccatccacctcactggccggtccctcctgccggcgctggaggccgagcccctctgggccaccgtctttggcagccagagccaccacgaggtcaccatgtcctaccccatgcgctccgtgcagcaccggcacttccgcctcgtgcacaacctcaacttcaagatgccctttcccatcgaccaggacttctacgtctcacccaccttccaggacctcctgaaccgcaccacagctggtcagcccacgggctggtacaaggacctccgtcattactactaccgggcgcgctgggagctctacgaccggagccgggacccccacgagacccagaacctggccaccgacccgcgctttgctcagcttctggagatgcttcgggaccagctggccaagtggcagtgggagacccacgacccctgggtgtgcgcccccgacggcgtcctggaggagaagctctctccccagtgccagcccctccacaatgagctgtaagcggccgc

SEQ ID NO: 277 - protein, 245 aa, Artificial Sequence
  Amino acid sequence of anti-hTfR single-chain antibody
EVQLVQSGAEVKKPGESLKISCKGSGYSFTNYWLGWVRQMPGKGLEWMGDIYPGGDYPTYSEKFKVQVTISADKSISTAYLQWSSLKASDTAMYYCARSGNYDEVAYWGQGTLVTVSSGGGGSGGGGSGGGGSDIVMTQTPLSLSVTPGQPASISCRSSQSLVHSNGNTYLHWYLQKPGQSPQLLIYKVSNRFSGVPDRFSGSGSGTDFTLKISRVEAEDVGVYYCSQSTHVPWTFGQGTKVEIK

SEQ ID NO: 278 - protein, 16 aa, Artificial Sequence
  Amino acid sequence 2 of CDR 2 in the heavy chain of mouse anti-hTfR antibody No. 6
IIWGDGSTNYHSALIS

SEQ ID NO: 279 - protein, 16 aa, Artificial Sequence
  Amino acid sequence 2 of CDR 2 in the heavy chain of mouse anti-hTfR antibody No. 8
IIWGDGSTNYRSALIS